European Patent Specification EP 4 110 387 B1, published May 21, 2025. Title: EX VIVO GAMMA DELTA T CELL POPULATIONS. Applicant: GammaDelta Therapeutics Limited. The sequence listing filed with the application follows.

SEQUENCE LISTING (338 sequences)

SEQ ID NO: 1 - protein, 256 aa, Homo sapiens
  V gamma 4 chain of RSCB Protein Data Bank entry: 4MNH
SSNLEGRTKSVIRQTGSSAEITCDLAEGSTGYIHWYLHQEGKAPQRLLYYDSYTSSVVLESGISPGKYDTYGSTRKNLRMILRNLIENDSGVYYCATWDEKYYKKLFGSGTTLVVTEDLKNVFPPEVAVFEPSEAEISHTQKATLVCLATGFYPDHVELSWWVNGKEVHSGVCTDPQPLKEQPALNDSRYALSSRLRVSATFWQNPRNHFRCQVQFYGLSENDEWTQDRAKPVTQIVSAEAWGRADSRGGLEVLFQ

SEQ ID NO: 2 - protein, 7 aa, artificial sequence
  G4_1 Heavy CDR3
GHWYFDL

SEQ ID NO: 3 - protein, 11 aa, artificial sequence
  G4_2 Heavy CDR3
FPVAGFYGMDV

SEQ ID NO: 4 - protein, 7 aa, artificial sequence
  G4_3 Heavy CDR3
GGWLYDY

SEQ ID NO: 5 - protein, 10 aa, artificial sequence
  G4_4 Heavy CDR3
SSVGWWSFDY

SEQ ID NO: 6 - protein, 11 aa, artificial sequence
  G4_5 Heavy CDR3
GGTGGDHVFAY

SEQ ID NO: 7 - protein, 11 aa, artificial sequence
  G4_6 Heavy CDR3
ADYGVVYYFDY

SEQ ID NO: 8 - protein, 10 aa, artificial sequence
  G4_7 Heavy CDR3
IGYSSSSFDY

SEQ ID NO: 9 - protein, 13 aa, artificial sequence
  G4_10 Heavy CDR3
DGAVDFWRNGMDV

SEQ ID NO: 10 - protein, 9 aa, artificial sequence
  G4_12 Heavy CDR3
VANGDFLDY

SEQ ID NO: 11 - protein, 8 aa, artificial sequence
  G4_13 Heavy CDR3
GGLGMVDP

SEQ ID NO: 12 - protein, 8 aa, artificial sequence
  G4_14 Heavy CDR3
DTAHGMDV

SEQ ID NO: 13 - protein, 13 aa, artificial sequence
  G4_15 Heavy CDR3
DNSHLDQVWWFDP

SEQ ID NO: 14 - protein, 10 aa, artificial sequence
  G4_16 Heavy CDR3
DYGDFYGMDV

SEQ ID NO: 15 - protein, 9 aa, artificial sequence
  G4_18 Heavy CDR3
DLDLSSLDY

SEQ ID NO: 16 - protein, 12 aa, artificial sequence
  G4_19 Heavy CDR3
ERGYSYGDGMDV

SEQ ID NO: 17 - protein, 10 aa, artificial sequence
  G4_20 Heavy CDR3
GNSRSDAFDI

SEQ ID NO: 18 - protein, 11 aa, artificial sequence
  G4_22 Heavy CDR3
DSTAVTDWFDP

SEQ ID NO: 19 - protein, 11 aa, artificial sequence
  G4_23 Heavy CDR3
GEVAALYYFDY

SEQ ID NO: 20 - protein, 10 aa, artificial sequence
  G4_24 Heavy CDR3
DWSSTRSFDY

SEQ ID NO: 21 - protein, 14 aa, artificial sequence
  G4_25 Heavy CDR3
SLRDGYNYIGSLGY

SEQ ID NO: 22 - protein, 11 aa, artificial sequence
  G4_26 Heavy CDR3
SRGSGWFPLGY

SEQ ID NO: 23 - protein, 13 aa, artificial sequence
  G4_27 Heavy CDR3
HGAYGDYPDTFDI

SEQ ID NO: 24 - protein, 16 aa, artificial sequence
  G4_28 Heavy CDR3
SYVDTAMRYYYYYMDV

SEQ ID NO: 25 - protein, 9 aa, artificial sequence
  G4_1 Light CDR3
QQSYSTPVT

SEQ ID NO: 26 - protein, 9 aa, artificial sequence
  G4_2 Light CDR3
LEDYNYLWT

SEQ ID NO: 27 - protein, 9 aa, artificial sequence
  G4_3 Light CDR3
QQSYSTPQT

SEQ ID NO: 28 - protein, 9 aa, artificial sequence
  G4_4 Light CDR3
QQYYSTPLT

SEQ ID NO: 29 - protein, 9 aa, artificial sequence
  G4_5 Light CDR3
QQSYSTPYT

SEQ ID NO: 30 - protein, 9 aa, artificial sequence
  G4_6 Light CDR3
QQSYSTPYT

SEQ ID NO: 31 - protein, 9 aa, artificial sequence
  G4_7 Light CDR3
MQGLQTPYT

SEQ ID NO: 32 - protein, 9 aa, artificial sequence
  G4_10 Light CDR3
MQGTLWPPT

SEQ ID NO: 33 - protein, 8 aa, artificial sequence
  G4_12 Light CDR3
SSHASPRV

SEQ ID NO: 34 - protein, 10 aa, artificial sequence
  G4_13 Light CDR3
QSYDSSIYVV

SEQ ID NO: 35 - protein, 10 aa, artificial sequence
  G4_14 Light CDR3
QSYDSSTHVV

SEQ ID NO: 36 - protein, 8 aa, artificial sequence
  G4_15 Light CDR3
SSYGSGSV

SEQ ID NO: 37 - protein, 10 aa, artificial sequence
  G4_16 Light CDR3
TSYAGSNTLI

SEQ ID NO: 38 - protein, 11 aa, artificial sequence
  G4_18 Light CDR3
QSADSSGTYTV

SEQ ID NO: 39 - protein, 10 aa, artificial sequence
  G4_19 Light CDR3
QSYDSSNHVV

SEQ ID NO: 40 - protein, 9 aa, artificial sequence
  G4_20 Light CDR3
QAWDSSTVV

SEQ ID NO: 41 - protein, 9 aa, artificial sequence
  G4_22 Light CDR3
QQSYSIPWT

SEQ ID NO: 42 - protein, 9 aa, artificial sequence
  G4_23 Light CDR3
QQYYSTPRT

SEQ ID NO: 43 - protein, 9 aa, artificial sequence
  G4_24 Light CDR3
QQYYSTPPT

SEQ ID NO: 44 - protein, 8 aa, artificial sequence
  G4_25 Light CDR3
SSYGSGSV

SEQ ID NO: 45 - protein, 8 aa, artificial sequence
  G4_26 Light CDR3
SSFGSGSI

SEQ ID NO: 46 - protein, 11 aa, artificial sequence
  G4_27 Light CDR3
NSRDSSGNHLV

SEQ ID NO: 47 - protein, 9 aa, artificial sequence
  G4_28 Light CDR3
NSRDSSGVV

SEQ ID NO: 48 - protein, 8 aa, artificial sequence
  G4_1 Heavy CDR2
ISSSSSYI

SEQ ID NO: 49 - protein, 8 aa, artificial sequence
  G4_2 Heavy CDR2
VDPEDGQS

SEQ ID NO: 50 - protein, 8 aa, artificial sequence
  G4_3 Heavy CDR2
ISSSSSYI

SEQ ID NO: 51 - protein, 8 aa, artificial sequence
  G4_4 Heavy CDR2
ISGSGGST

SEQ ID NO: 52 - protein, 8 aa, artificial sequence
  G4_5 Heavy CDR2
IGAYNGNT

SEQ ID NO: 53 - protein, 8 aa, artificial sequence
  G4_6 Heavy CDR2
ISGSGGST

SEQ ID NO: 54 - protein, 8 aa, artificial sequence
  G4_7 Heavy CDR2
IKQDGSII

SEQ ID NO: 55 - protein, 8 aa, artificial sequence
  G4_10 Heavy CDR2
ISGSGGST

SEQ ID NO: 56 - protein, 7 aa, artificial sequence
  G4_12 Heavy CDR2
IYSGGST

SEQ ID NO: 57 - protein, 8 aa, artificial sequence
  G4_13 Heavy CDR2
ISGTSSYI

SEQ ID NO: 58 - protein, 8 aa, artificial sequence
  G4_14 Heavy CDR2
IDPSDSYT

SEQ ID NO: 59 - protein, 8 aa, artificial sequence
  G4_15 Heavy CDR2
INPSGSST

SEQ ID NO: 60 - protein, 8 aa, artificial sequence
  G4_16 Heavy CDR2
ISAYNGNT

SEQ ID NO: 61 - protein, 8 aa, artificial sequence
  G4_18 Heavy CDR2
INPNSGGT

SEQ ID NO: 62 - protein, 8 aa, artificial sequence
  G4_19 Heavy CDR2
INPSGGST

SEQ ID NO: 63 - protein, 8 aa, artificial sequence
  G4_20 Heavy CDR2
IIPIFGTA

SEQ ID NO: 64 - protein, 8 aa, artificial sequence
  G4_22 Heavy CDR2
VSGSGGTT

SEQ ID NO: 65 - protein, 8 aa, artificial sequence
  G4_23 Heavy CDR2
IWYDGSNK

SEQ ID NO: 66 - protein, 9 aa, artificial sequence
  G4_24 Heavy CDR2
TYYRSRWYN

SEQ ID NO: 67 - protein, 8 aa, artificial sequence
  G4_25 Heavy CDR2
IIPIFGTA

SEQ ID NO: 68 - protein, 8 aa, artificial sequence
  G4_26 Heavy CDR2
IIPIFGTA

SEQ ID NO: 69 - protein, 8 aa, artificial sequence
  G4_27 Heavy CDR2
IYPGDSDT

SEQ ID NO: 70 - protein, 8 aa, artificial sequence
  G4_28 Heavy CDR2
ISAGGGST

SEQ ID NO: 71 - protein, 8 aa, artificial sequence
  G4_1 Heavy CDR1
GFTFSSYS

SEQ ID NO: 72 - protein, 8 aa, artificial sequence
  G4_2 Heavy CDR1
GYPFTDYY

SEQ ID NO: 73 - protein, 8 aa, artificial sequence
  G4_3 Heavy CDR1
GFTFSSYS

SEQ ID NO: 74 - protein, 8 aa, artificial sequence
  G4_4 Heavy CDR1
GFTFSSYA

SEQ ID NO: 75 - protein, 8 aa, artificial sequence
  G4_5 Heavy CDR1
GYTFTSYG

SEQ ID NO: 76 - protein, 8 aa, artificial sequence
  G4_6 Heavy CDR1
GFTFSSYA

SEQ ID NO: 77 - protein, 8 aa, artificial sequence
  G4_7 Heavy CDR1
GFTFSHYW

SEQ ID NO: 78 - protein, 8 aa, artificial sequence
  G4_10 Heavy CDR1
GFTFSSYA

SEQ ID NO: 79 - protein, 8 aa, artificial sequence
  G4_12 Heavy CDR1
GFTVSSNY

SEQ ID NO: 80 - protein, 8 aa, artificial sequence
  G4_13 Heavy CDR1
GFTFSSYS

SEQ ID NO: 81 - protein, 8 aa, artificial sequence
  G4_14 Heavy CDR1
GYSFTSYW

SEQ ID NO: 82 - protein, 8 aa, artificial sequence
  G4_15 Heavy CDR1
GYTFTRHY

SEQ ID NO: 83 - protein, 8 aa, artificial sequence
  G4_16 Heavy CDR1
GYTFTSYG

SEQ ID NO: 84 - protein, 8 aa, artificial sequence
  G4_18 Heavy CDR1
GYTFTGYY

SEQ ID NO: 85 - protein, 8 aa, artificial sequence
  G4_19 Heavy CDR1
GYTLTSYY

SEQ ID NO: 86 - protein, 8 aa, artificial sequence
  G4_20 Heavy CDR1
GGTFSSYA

SEQ ID NO: 87 - protein, 8 aa, artificial sequence
  G4_22 Heavy CDR1
GFTFSTYA

SEQ ID NO: 88 - protein, 8 aa, artificial sequence
  G4_23 Heavy CDR1
GFTFSSYG

SEQ ID NO: 89 - protein, 10 aa, artificial sequence
  G4_24 Heavy CDR1
GASVSSNSVA

SEQ ID NO: 90 - protein, 8 aa, artificial sequence
  G4_25 Heavy CDR1
GGTFSSYA

SEQ ID NO: 91 - protein, 8 aa, artificial sequence
  G4_26 Heavy CDR1
GGTFSSYA

SEQ ID NO: 92 - protein, 8 aa, artificial sequence
  G4_27 Heavy CDR1
GYSFTSYW

SEQ ID NO: 93 - protein, 8 aa, artificial sequence
  G4_28 Heavy CDR1
GFTFDDYA

SEQ ID NO: 94 - protein, 6 aa, artificial sequence
  G4_1 Light CDR1
QDISNY

SEQ ID NO: 95 - protein, 6 aa, artificial sequence
  G4_2 Light CDR1
QDISNY

SEQ ID NO: 96 - protein, 6 aa, artificial sequence
  G4_3 Light CDR1
QDISNY

SEQ ID NO: 97 - protein, 12 aa, artificial sequence
  G4_4 Light CDR1
QSVLSSSNNNNY

SEQ ID NO: 98 - protein, 6 aa, artificial sequence
  G4_5 Light CDR1
QSISSY

SEQ ID NO: 99 - protein, 6 aa, artificial sequence
  G4_6 Light CDR1
QSISTY

SEQ ID NO: 100 - protein, 11 aa, artificial sequence
  G4_7 Light CDR1
QSLLHSNRFNY

SEQ ID NO: 101 - protein, 11 aa, artificial sequence
  G4_10 Light CDR1
QSLEYSDGNTY

SEQ ID NO: 102 - protein, 9 aa, artificial sequence
  G4_12 Light CDR1
SSDVGGYNF

SEQ ID NO: 103 - protein, 8 aa, artificial sequence
  G4_13 Light CDR1
SGSIASNY

SEQ ID NO: 104 - protein, 8 aa, artificial sequence
  G4_14 Light CDR1
RGSIAGNY

SEQ ID NO: 105 - protein, 9 aa, artificial sequence
  G4_15 Light CDR1
SSDVGGYNY

SEQ ID NO: 106 - protein, 9 aa, artificial sequence
  G4_16 Light CDR1
SSDIGAFNS

SEQ ID NO: 107 - protein, 6 aa, artificial sequence
  G4_18 Light CDR1
ALAKQY

SEQ ID NO: 108 - protein, 8 aa, artificial sequence
  G4_19 Light CDR1
SGSIASNY

SEQ ID NO: 109 - protein, 6 aa, artificial sequence
  G4_20 Light CDR1
KLGDKF

SEQ ID NO: 110 - protein, 6 aa, artificial sequence
  G4_22 Light CDR1
QDISNY

SEQ ID NO: 111 - protein, 6 aa, artificial sequence
  G4_23 Light CDR1
QGISNS

SEQ ID NO: 112 - protein, 12 aa, artificial sequence
  G4_24 Light CDR1
QSVLYSSNNKNY

SEQ ID NO: 113 - protein, 9 aa, artificial sequence
  G4_25 Light CDR1
SSDVGGYNY

SEQ ID NO: 114 - protein, 9 aa, artificial sequence
  G4_26 Light CDR1
SSDVGSYNL

SEQ ID NO: 115 - protein, 6 aa, artificial sequence
  G4_27 Light CDR1
SLRNFY

SEQ ID NO: 116 - protein, 6 aa, artificial sequence
  G4_28 Light CDR1
SLRNYY

SEQ ID NO: 117 - protein, 116 aa, artificial sequence
  TRGV4 full heavy variable sequence G4_1
EVQLLESGGGVVQPGRPLRLSCAASGFTFSSYSMNWVRQAPGKGLEWVSSISSSSSYIYYADSVKGRFTISRDNSKNTLYLQMNSLRAEDTAVYYCAKGHWYFDLWGRGTLVTVSS

SEQ ID NO: 118 - protein, 120 aa, artificial sequence
  TRGV4 full heavy variable sequence G4_2
QMQLVQSGAEVKKPGATVKISCKVSGYPFTDYYIHWVQQAPGKGLEWMGLVDPEDGQSRSAERFQGRVTITADTSTDTAYMELSSLRSEDTAVYYCATFPVAGFYGMDVWGQGTLVTVSS

SEQ ID NO: 119 - protein, 116 aa, artificial sequence
  TRGV4 full heavy variable sequence G4_3
EVQLVESGGGLVQPGGSLRLSCAASGFTFSSYSMNWVRQAPGKGLEWVSSISSSSSYIYYADSVKGRFTISRDNSKNTLYLQMNSLRAEDTAVYYCARGGWLYDYWGQGTLVTVSS

SEQ ID NO: 120 - protein, 119 aa, artificial sequence
  TRGV4 full heavy variable sequence G4_4
QVQLVESGGGLVQPGGSLRLSCAASGFTFSSYAMSWVRQAPGKGLEWVSAISGSGGSTYYADSVKGRFTISRDNSKNTLYLQMSSLRVEDTAVYYCAKSSVGWWSFDYWGQGTMVTVSS

SEQ ID NO: 121 - protein, 120 aa, artificial sequence
  TRGV4 full heavy variable sequence G4_5
EVQLVQSGAEVKKPGSSVKVSCKASGYTFTSYGISWVRQAPGQGLEWMGWIGAYNGNTNYAQKLQGRVTMSTDTSTSTAYMELRSPRSDDTAVYYCARGGTGGDHVFAYWGQGTTVTVSS

SEQ ID NO: 122 - protein, 120 aa, artificial sequence
  TRGV4 full heavy variable sequence G4_6
EVQLVESGGGLVQPGGPLRLSCAASGFTFSSYAMNWVRQAPGKGLEWVSAISGSGGSTYYADSVKGRFTISRDNSKNTLYLQMNSLRAEDTAVYYCAKADYGVVYYFDYWGQGTMVTVSS

SEQ ID NO: 123 - protein, 119 aa, artificial sequence
  TRGV4 full heavy variable sequence G4_7
EVQLVESGGGWVQSGGSLRPSCAASGFTFSHYWMSWVRQAPGKGLEWVANIKQDGSIIYYADSVKGRFTISRDNAKNSVYLQMNSLRAEDTAVYYCARIGYSSSSFDYWGRGTLVTVSS

SEQ ID NO: 124 - protein, 122 aa, artificial sequence
  TRGV4 full heavy variable sequence G4_10
QVQLVESGGGVVQPGRPLRLSCAASGFTFSSYAMHWVRQAPGKGLEWVSAISGSGGSTYYADSVKGRFTISRDNSKNTLYLQMNSLRAEDTAVYYCAKDGAVDFWRNGMDVWGRGTLVTVSS

SEQ ID NO: 125 - protein, 117 aa, artificial sequence
  TRGV4 full heavy variable sequence G4_12
EVQLLESGGGLVQPGGSLRLSCAASGFTVSSNYMSWVRQAPGKGLEWVSVIYSGGSTYYADSVKGRFTISRHNSKNTLYLQMNSLRAEDTAVYYCARVANGDFLDYWGRGTLVTVSS

SEQ ID NO: 126 - protein, 117 aa, artificial sequence
  TRGV4 full heavy variable sequence G4_13
QVQLVESGAEVKKPGGSLRLSCAASGFTFSSYSMNWVRQAPGKGLEWVSSISGTSSYIYYADSVKGRFTISRDNAKNSLYLQMSSLRAEDTAVYYCARGGLGMVDPWGQGTLVTVSS

SEQ ID NO: 127 - protein, 117 aa, artificial sequence
  TRGV4 full heavy variable sequence G4_14
EVQLVQSGAEVKKPGESLRISCKGSGYSFTSYWISWVRQMPGKGLEWMGRIDPSDSYTNYSPSFPGHVTISADKSISTAYLQWSSLKASDTAMYYCAADTAHGMDVWGRGTLVTVSS

SEQ ID NO: 128 - protein, 122 aa, artificial sequence
  TRGV4 full heavy variable sequence G4_15
EVQLVQSEAEVKKPGASVKVSCKASGYTFTRHYMHWVRQAPGQGLEWMGLINPSGSSTVYAQKFQGRVTLTRDTSTSTDYMELSSLRSEDTAVYYCARDNSHLDQVWWFDPWGQGTLVTVSS

SEQ ID NO: 129 - protein, 119 aa, artificial sequence
  TRGV4 full heavy variable sequence G4_16
EVQLLESGAEVKKPGASVKVSCKASGYTFTSYGISWVRQAPGQGLEWMGWISAYNGNTNYAQKLQGRVTMTTDTSTSTAYMELRSLRSDDTAVYYCARDYGDFYGMDVWGQGTLVTVSS

SEQ ID NO: 130 - protein, 118 aa, artificial sequence
  TRGV4 full heavy variable sequence G4_18
EVQLVESGAEVKKPGASVKVSCKASGYTFTGYYMHWVRQAPGQGLEWMGRINPNSGGTNYAQKFQGRVTMTRDASISTAYMELSRLRSDDTAVYYCARDLDLSSLDYWGRGTLVTVSS

SEQ ID NO: 131 - protein, 121 aa, artificial sequence
  TRGV4 full heavy variable sequence G4_19
EVQLVQSGAEVKKPGASVKVSCKASGYTLTSYYMHWVRQAPGQGLEWMGIINPSGGSTSYAQKFQGRVTMTRDTSTSTVYMELSSLRSEDTAVYYCARERGYSYGDGMDVWGQGTTVTVSS

SEQ ID NO: 132 - protein, 119 aa, artificial sequence
  TRGV4 full heavy variable sequence G4_20
QVQLVESGAEVKKPGASVKVSCKASGGTFSSYAISWVRQAPGQGLEWMGGIIPIFGTANYAQKFQGRVTITVDKSTRTAYMELSSLRSKDTAVYYCARGNSRSDAFDIWGQGTMVTVSS

SEQ ID NO: 133 - protein, 120 aa, artificial sequence
  TRGV4 full heavy variable sequence G4_22
QVQLVESGGGLVQPGGSLRLSCAASGFTFSTYAMSWVRQAPGKGLEWVSTVSGSGGTTYYADSVKGRFTISRDNSKNTLYLQMNSLRAEDTAVYYCAKDSTAVTDWFDPWGRGTLVTVSS

SEQ ID NO: 134 - protein, 120 aa, artificial sequence
  TRGV4 full heavy variable sequence G4_23
EVQLVESGGGVVQPGRSLRLSCAASGFTFSSYGMHWVRQAPGKGLEWVAVIWYDGSNKYYADSVKGRFTISRDNSKNTLYLQMNSLRAEDTAVYYCARGEVAALYYFDYWGQGTLVTVSS

SEQ ID NO: 135 - protein, 122 aa, artificial sequence
  TRGV4 full heavy variable sequence G4_24
QVQLQQSGPGLVKPSQTLSLTCAISGASVSSNSVAWNWIRQSPSRGLEWLGRTYYRSRWYNDYALSVKSRIIINPDTSKNQFSLQLNSVTPEDTAVYYCARDWSSTRSFDYWGRGTLVTVSS

SEQ ID NO: 136 - protein, 123 aa, artificial sequence
  TRGV4 full heavy variable sequence G4_25
EVQLVESGAEVKKPGSSVKVSCKASGGTFSSYAISWVRQAPGQGLEWMGGIIPIFGTANYAQKFQGRVTITADKSTSTAYMELSSLRSEDTAVYYCARSLRDGYNYIGSLGYWGQGTLVTVSS

SEQ ID NO: 137 - protein, 120 aa, artificial sequence
  TRGV4 full heavy variable sequence G4_26
QVQLVQSGAEVKKPGSSVKVSCKASGGTFSSYAISWVRQAPGQGLEWMGGIIPIFGTANYAQKFQGRVTITADESTSTAYMELSSLRSEDTAVYYCASSRGSGWFPLGYWGQGTLVTVSS

SEQ ID NO: 138 - protein, 122 aa, artificial sequence
  TRGV4 full heavy variable sequence G4_27
QVQLVQSGAEVKKPGESLKISCKSSGYSFTSYWIGWVRQMPGKGLEWMGIIYPGDSDTRYSPSFQGQVTFSADESISTAYLQWSSLKASDTAMYYCARHGAYGDYPDTFDIWGQGTLVTVSS

SEQ ID NO: 139 - protein, 125 aa, artificial sequence
  TRGV4 full heavy variable sequence G4_28
QVQLVESGGGLVQPGGSLRLSCAASGFTFDDYAMHWVRQAPGKGLEWVSGISAGGGSTNYAGSVKGRFTVSRDTSKNTLYLQMNSLRAEDTAVYYCVKSYVDTAMRYYYYYMDVWGQGTMVTVSS

SEQ ID NO: 140 - protein, 109 aa, artificial sequence
  TRGV4 full light variable sequence G4_1
ASDIQMTQSPSSLSASVGDRVTITCQASQDISNYLNWYQQKPGKAPKLLIYDASNLETGVPSRFSGSGSGTDFTLTISSLQPEDFATYYCQQSYSTPVTFGPGTKVEIK

SEQ ID NO: 141 - protein, 109 aa, artificial sequence
  TRGV4 full light variable sequence G4_2
ASDIQMTQSPSSLSASVGDRVTITCQASQDISNYLNWYQQKPGKAPKLLIYAASSLQSGVPSRFSGSGSGTDFTLTISGLQPEDFATYYCLEDYNYLWTFGQGTKLEIK

SEQ ID NO: 142 - protein, 109 aa, artificial sequence
  TRGV4 full light variable sequence G4_3
ASDIQMTQSPSSLSASVGDRVTITCQASQDISNYLNWYQQKPGKAPKLLIYDASNLETGVPSRFSGSGSGTDFTLTISSLQPEDFATYFCQQSYSTPQTFGQGTKVDIK

SEQ ID NO: 143 - protein, 115 aa, artificial sequence
  TRGV4 full light variable sequence G4_4
ASDIVMTQSPDSLAVSLGERATINCKSSQSVLSSSNNNNYLAWYQQRPGQPPKLLFYWASTRESGVPDRFSGSGSGTSFTLTITSLQAEDVAVYYCQQYYSTPLTFGGGTKLEIK

SEQ ID NO: 144 - protein, 109 aa, artificial sequence
  TRGV4 full light variable sequence G4_5
ASDIQMTQSPSSLSASVGDRVTITCRASQSISSYLNWYQQKPGKAPKLLIYAASSLQSGVPSRFSGSGSGTDFTLTISSLQPEDFATYYCQQSYSTPYTFGQGTKVEIK

SEQ ID NO: 145 - protein, 109 aa, artificial sequence
  TRGV4 full light variable sequence G4_6
ASDIQMTQSPSSLSASVGDRVTITCRASQSISTYLNWYQQKPGKAPKLLIYAASSLQSGVPSRFSGSGSGTDFTLTISSPQPEDFATYYCQQSYSTPYTFGQGTKVEIK

SEQ ID NO: 146 - protein, 114 aa, artificial sequence
  TRGV4 full light variable sequence G4_7
ASDIVMTQSPLSLPVTPGEPASISCRSSQSLLHSNRFNYLDWYLQKPGQSPQLLIYLGSNRASGVPDRFSGSGSGTDFTLKISRVEAEDVGVYYCMQGLQTPYTFGQGTKVDIK

SEQ ID NO: 147 - protein, 114 aa, artificial sequence
  TRGV4 full light variable sequence G4_10
ASDIVMTQPPLSLPVTLGHPASISCKSSQSLEYSDGNTYLNWFQQRPGQSPRRLIYKVSNRDSGAPDRFSGSGSGTDFTLEISRVEAEDVGVYYCMQGTLWPPTFGQGTKVDIK

SEQ ID NO: 148 - protein, 110 aa, artificial sequence
  TRGV4 full light variable sequence G4_12
ASQSVLTQPASVSGSPGQSITISCTGTSSDVGGYNFVSWYQQHPGKAPKLMIYEVTNRPSGVPDRFSGSKSGNTASLTISGLQAEDEADYYCSSHASPRVFGTGTKVTVL

SEQ ID NO: 149 - protein, 113 aa, artificial sequence
  TRGV4 full light variable sequence G4_13
ASNFMLTQPHSVSESPGKTVTISCTRSSGSIASNYVQWYQQRPGSSPSTVIYEDNQRPSGVPDRFSGSIDSSSNSASLTISGLRTEDEADYYCQSYDSSIYVVFGGGTKLTVL

SEQ ID NO: 150 - protein, 113 aa, artificial sequence
  TRGV4 full light variable sequence G4_14
ASNFMLTQPHSVSESPGKTVTISCTRSRGSIAGNYVHWYQQRPGRAPTTVIYRDKERPSGVPDRISGSIDSSSNSASLTISGLKTEDEADYYCQSYDSSTHVVFGGGTKLTVL

SEQ ID NO: 151 - protein, 110 aa, artificial sequence
  TRGV4 full light variable sequence G4_15
ASQSALTQPASVSGSPGQSITISCTGTSSDVGGYNYVSWYQQHPGKAPKLMIYDVSNRPSGVSNRFSGSKSGNTASLTISGLQAEDEADYYCSSYGSGSVFGTGTKLTVL

SEQ ID NO: 152 - protein, 112 aa, artificial sequence
  TRGV4 full light variable sequence G4_16
ASQSVLTQPPSASGSPGQSVTFSCTGTSSDIGAFNSVSWYQQHPGKAPKLLIYEITKRPSGVPDRFSGSKSGNTASLTISVLQAEDEADYYCTSYAGSNTLIFGGGTKVTVL

SEQ ID NO: 153 - protein, 110 aa, artificial sequence
  TRGV4 full light variable sequence G4_18
ASSYELTQPPSVTESPGQTARITCSGDALAKQYAYWYQQKPGQAPVLVIYRDSERPSEIPERFSGSSSGTTVTLTISGVQAEDEADYYCQSADSSGTYTVFGGGTKLTVL

SEQ ID NO: 154 - protein, 113 aa, artificial sequence
  TRGV4 full light variable sequence G4_19
ASNFMLTQPHSVSESPGKTVTISCTRSSGSIASNYVQWYQQRPGSPPITLIYDDDQRPSGVPHRFSGSIDTSSNPASLTISGLKTEDEADYYCQSYDSSNHVVFGGGTKLTVL

SEQ ID NO: 155 - protein, 108 aa, artificial sequence
  TRGV4 full light variable sequence G4_20
ASSYELTHPPSVSVSPGQTASITCSGDKLGDKFVSWYHQKPGQSPVLVIYQDSKRPSGIPERFSGSNSGNTATLTISGTRAMDEADYYCQAWDSSTVVFGGGTKLTVL

SEQ ID NO: 156 - protein, 109 aa, artificial sequence
  TRGV4 full light variable sequence G4_22
ASDIQMTQSPSSLSASVGDRVTITCQASQDISNYLNWYQQKPGKAPKLLIYAASSLQSGVPSRFSVSGSGTDFTLTISNLQPEDFATYYCQQSYSIPWTFGQGTKVEIK

SEQ ID NO: 157 - protein, 109 aa, artificial sequence
  TRGV4 full light variable sequence G4_23
ASDIQMTQSPSSLSASVGDRVTITCRASQGISNSLAWYQQKPGKAPKLLLYAASRLESGVPSRFSGSGSGTDYTLTISSLQPEDFATYYCQQYYSTPRTFGGGTKLEIK

SEQ ID NO: 158 - protein, 115 aa, artificial sequence
  TRGV4 full light variable sequence G4_24
ASDIVMTQSPDSLAVSLGERATINCKSSQSVLYSSNNKNYLAWYQQKPGQPPKLLISWASTRESGVPDRFSGSGSGTDFTLTINSLQSEDVAIYYCQQYYSTPPTFGQGTKLEIK

SEQ ID NO: 159 - protein, 110 aa, artificial sequence
  TRGV4 full light variable sequence G4_25
ASQSALTQPRSVSGSPGQSVTISCTGTSSDVGGYNYVSWYQQHPGKAPKLMIYEVSNRPSGVSNRFSGSKSGNTASLTISGLQAEDEADYYCSSYGSGSVFGTGTKLTVL

SEQ ID NO: 160 - protein, 110 aa, artificial sequence
  TRGV4 full light variable sequence G4_26
ASQSGLTQPASVSGSPGQSITISCTGTSSDVGSYNLVSWYQQHPGKAPKLMIYEVSKRPSGVSNRFSGSKSGNTASLTISGLQAEDEADYYCSSFGSGSIFGTGTKLTVL

SEQ ID NO: 161 - protein, 110 aa, artificial sequence
  TRGV4 full light variable sequence G4_27
ASSYELTQDPAVSVALGQTVSITCQGDSLRNFYANWYQQKPGQAPVLVIYGKNNRPSGIPDRFSGSSSGNTASLTITGAQAEDEADYYCNSRDSSGNHLVFGGGTQLTVL

SEQ ID NO: 162 - protein, 108 aa, artificial sequence
  TRGV4 full light variable sequence G4_28
ASSYELTQDPAVSVALGQTVTITCQGDSLRNYYASWYRQKPGQTPVLVVYGKNNRPSGIPDRFSVSASGNTASLTITGAQAEDEGDYYCNSRDSSGVVFGGGTKVTVL

SEQ ID NO: 163 - protein, 275 aa, artificial sequence
  scFv sequence G4_1
EVQLLESGGGVVQPGRPLRLSCAASGFTFSSYSMNWVRQAPGKGLEWVSSISSSSSYIYYADSVKGRFTISRDNSKNTLYLQMNSLRAEDTAVYYCAKGHWYFDLWGRGTLVTVSSGGGGSGGGGSGGGASDIQMTQSPSSLSASVGDRVTITCQASQDISNYLNWYQQKPGKAPKLLIYDASNLETGVPSRFSGSGSGTDFTLTISSLQPEDFATYYCQQSYSTPVTFGPGTKVEIKRTAAASAHHHHHHKLDYKDHDGDYKDHDIDYKDDDDK

SEQ ID NO: 164 - protein, 279 aa, artificial sequence
  scFv sequence G4_2
QMQLVQSGAEVKKPGATVKISCKVSGYPFTDYYIHWVQQAPGKGLEWMGLVDPEDGQSRSAERFQGRVTITADTSTDTAYMELSSLRSEDTAVYYCATFPVAGFYGMDVWGQGTLVTVSSGGGGSGGGGSGGGASDIQMTQSPSSLSASVGDRVTITCQASQDISNYLNWYQQKPGKAPKLLIYAASSLQSGVPSRFSGSGSGTDFTLTISGLQPEDFATYYCLEDYNYLWTFGQGTKLEIKRTAAASAHHHHHHKLDYKDHDGDYKDHDIDYKDDDDK

SEQ ID NO: 165 - protein, 275 aa, artificial sequence
  scFv sequence G4_3
EVQLVESGGGLVQPGGSLRLSCAASGFTFSSYSMNWVRQAPGKGLEWVSSISSSSSYIYYADSVKGRFTISRDNSKNTLYLQMNSLRAEDTAVYYCARGGWLYDYWGQGTLVTVSSGGGGSGGGGSGGGASDIQMTQSPSSLSASVGDRVTITCQASQDISNYLNWYQQKPGKAPKLLIYDASNLETGVPSRFSGSGSGTDFTLTISSLQPEDFATYFCQQSYSTPQTFGQGTKVDIKRTAAASAHHHHHHKLDYKDHDGDYKDHDIDYKDDDDK

SEQ ID NO: 166 - protein, 284 aa, artificial sequence
  scFv sequence G4_4
QVQLVESGGGLVQPGGSLRLSCAASGFTFSSYAMSWVRQAPGKGLEWVSAISGSGGSTYYADSVKGRFTISRDNSKNTLYLQMSSLRVEDTAVYYCAKSSVGWWSFDYWGQGTMVTVSSGGGGSGGGGSGGGASDIVMTQSPDSLAVSLGERATINCKSSQSVLSSSNNNNYLAWYQQRPGQPPKLLFYWASTRESGVPDRFSGSGSGTSFTLTITSLQAEDVAVYYCQQYYSTPLTFGGGTKLEIKRTAAASAHHHHHHKLDYKDHDGDYKDHDIDYKDDDDK

SEQ ID NO: 167 - protein, 279 aa, artificial sequence
  scFv sequence G4_5
EVQLVQSGAEVKKPGSSVKVSCKASGYTFTSYGISWVRQAPGQGLEWMGWIGAYNGNTNYAQKLQGRVTMSTDTSTSTAYMELRSPRSDDTAVYYCARGGTGGDHVFAYWGQGTTVTVSSGGGGSGGGGSGGGASDIQMTQSPSSLSASVGDRVTITCRASQSISSYLNWYQQKPGKAPKLLIYAASSLQSGVPSRFSGSGSGTDFTLTISSLQPEDFATYYCQQSYSTPYTFGQGTKVEIKRTAAASAHHHHHHKLDYKDHDGDYKDHDIDYKDDDDK

SEQ ID NO: 168 - protein, 279 aa, artificial sequence
  scFv sequence G4_6
EVQLVESGGGLVQPGGPLRLSCAASGFTFSSYAMNWVRQAPGKGLEWVSAISGSGGSTYYADSVKGRFTISRDNSKNTLYLQMNSLRAEDTAVYYCAKADYGVVYYFDYWGQGTMVTVSSGGGGSGGGGSGGGASDIQMTQSPSSLSASVGDRVTITCRASQSISTYLNWYQQKPGKAPKLLIYAASSLQSGVPSRFSGSGSGTDFTLTISSPQPEDFATYYCQQSYSTPYTFGQGTKVEIKRTAAASAHHHHHHKLDYKDHDGDYKDHDIDYKDDDDK

SEQ ID NO: 169 - protein, 283 aa, artificial sequence
  scFv sequence G4_7
EVQLVESGGGWVQSGGSLRPSCAASGFTFSHYWMSWVRQAPGKGLEWVANIKQDGSIIYYADSVKGRFTISRDNAKNSVYLQMNSLRAEDTAVYYCARIGYSSSSFDYWGRGTLVTVSSGGGGSGGGGSGGGASDIVMTQSPLSLPVTPGEPASISCRSSQSLLHSNRFNYLDWYLQKPGQSPQLLIYLGSNRASGVPDRFSGSGSGTDFTLKISRVEAEDVGVYYCMQGLQTPYTFGQGTKVDIKRTAAASAHHHHHHKLDYKDHDGDYKDHDIDYKDDDDK

SEQ ID NO: 170 - protein, 286 aa, artificial sequence
  scFv sequence G4_10
QVQLVESGGGVVQPGRPLRLSCAASGFTFSSYAMHWVRQAPGKGLEWVSAISGSGGSTYYADSVKGRFTISRDNSKNTLYLQMNSLRAEDTAVYYCAKDGAVDFWRNGMDVWGRGTLVTVSSGGGGSGGGGSGGGASDIVMTQPPLSLPVTLGHPASISCKSSQSLEYSDGNTYLNWFQQRPGQSPRRLIYKVSNRDSGAPDRFSGSGSGTDFTLEISRVEAEDVGVYYCMQGTLWPPTFGQGTKVDIKRTAAASAHHHHHHKLDYKDHDGDYKDHDIDYKDDDDK

SEQ ID NO: 171 - protein, 277 aa, artificial sequence
  scFv sequence G4_12
EVQLLESGGGLVQPGGSLRLSCAASGFTVSSNYMSWVRQAPGKGLEWVSVIYSGGSTYYADSVKGRFTISRHNSKNTLYLQMNSLRAEDTAVYYCARVANGDFLDYWGRGTLVTVSSGGGGSGGGGSGGGASQSVLTQPASVSGSPGQSITISCTGTSSDVGGYNFVSWYQQHPGKAPKLMIYEVTNRPSGVPDRFSGSKSGNTASLTISGLQAEDEADYYCSSHASPRVFGTGTKVTVLRTAAASAHHHHHHKLDYKDHDGDYKDHDIDYKDDDDK

SEQ ID NO: 172 - protein, 280 aa, artificial sequence
  scFv sequence G4_13
QVQLVESGAEVKKPGGSLRLSCAASGFTFSSYSMNWVRQAPGKGLEWVSSISGTSSYIYYADSVKGRFTISRDNAKNSLYLQMSSLRAEDTAVYYCARGGLGMVDPWGQGTLVTVSSGGGGSGGGGSGGGASNFMLTQPHSVSESPGKTVTISCTRSSGSIASNYVQWYQQRPGSSPSTVIYEDNQRPSGVPDRFSGSIDSSSNSASLTISGLRTEDEADYYCQSYDSSIYVVFGGGTKLTVLRTAAASAHHHHHHKLDYKDHDGDYKDHDIDYKDDDDK

SEQ ID NO: 173 - protein, 280 aa, artificial sequence
  scFv sequence G4_14
EVQLVQSGAEVKKPGESLRISCKGSGYSFTSYWISWVRQMPGKGLEWMGRIDPSDSYTNYSPSFPGHVTISADKSISTAYLQWSSLKASDTAMYYCAADTAHGMDVWGRGTLVTVSSGGGGSGGGGSGGGASNFMLTQPHSVSESPGKTVTISCTRSRGSIAGNYVHWYQQRPGRAPTTVIYRDKERPSGVPDRISGSIDSSSNSASLTISGLKTEDEADYYCQSYDSSTHVVFGGGTKLTVLRTAAASAHHHHHHKLDYKDHDGDYKDHDIDYKDDDDK

SEQ ID NO: 174 - protein, 282 aa, artificial sequence
  scFv sequence G4_15
EVQLVQSEAEVKKPGASVKVSCKASGYTFTRHYMHWVRQAPGQGLEWMGLINPSGSSTVYAQKFQGRVTLTRDTSTSTDYMELSSLRSEDTAVYYCARDNSHLDQVWWFDPWGQGTLVTVSSGGGGSGGGGSGGGASQSALTQPASVSGSPGQSITISCTGTSSDVGGYNYVSWYQQHPGKAPKLMIYDVSNRPSGVSNRFSGSKSGNTASLTISGLQAEDEADYYCSSYGSGSVFGTGTKLTVLRTAAASAHHHHHHKLDYKDHDGDYKDHDIDYKDDDDK

SEQ ID NO: 175 - protein, 281 aa, artificial sequence
  scFv sequence G4_16
EVQLLESGAEVKKPGASVKVSCKASGYTFTSYGISWVRQAPGQGLEWMGWISAYNGNTNYAQKLQGRVTMTTDTSTSTAYMELRSLRSDDTAVYYCARDYGDFYGMDVWGQGTLVTVSSGGGGSGGGGSGGGASQSVLTQPPSASGSPGQSVTFSCTGTSSDIGAFNSVSWYQQHPGKAPKLLIYEITKRPSGVPDRFSGSKSGNTASLTISVLQAEDEADYYCTSYAGSNTLIFGGGTKVTVLRTAAASAHHHHHHKLDYKDHDGDYKDHDIDYKDDDDK

SEQ ID NO: 176 - protein, 278 aa, artificial sequence
  scFv sequence G4_18
EVQLVESGAEVKKPGASVKVSCKASGYTFTGYYMHWVRQAPGQGLEWMGRINPNSGGTNYAQKFQGRVTMTRDASISTAYMELSRLRSDDTAVYYCARDLDLSSLDYWGRGTLVTVSSGGGGSGGGGSGGGASSYELTQPPSVTESPGQTARITCSGDALAKQYAYWYQQKPGQAPVLVIYRDSERPSEIPERFSGSSSGTTVTLTISGVQAEDEADYYCQSADSSGTYTVFGGGTKLTVLRTAAASAHHHHHHKLDYKDHDGDYKDHDIDYKDDDDK

SEQ ID NO: 177 - protein, 284 aa, artificial sequence
  scFv sequence G4_19
EVQLVQSGAEVKKPGASVKVSCKASGYTLTSYYMHWVRQAPGQGLEWMGIINPSGGSTSYAQKFQGRVTMTRDTSTSTVYMELSSLRSEDTAVYYCARERGYSYGDGMDVWGQGTTVTVSSGGGGSGGGGSGGGASNFMLTQPHSVSESPGKTVTISCTRSSGSIASNYVQWYQQRPGSPPITLIYDDDQRPSGVPHRFSGSIDTSSNPASLTISGLKTEDEADYYCQSYDSSNHVVFGGGTKLTVLRTAAASAHHHHHHKLDYKDHDGDYKDHDIDYKDDDDK

SEQ ID NO: 178 - protein, 277 aa, artificial sequence
  scFv sequence G4_20
QVQLVESGAEVKKPGASVKVSCKASGGTFSSYAISWVRQAPGQGLEWMGGIIPIFGTANYAQKFQGRVTITVDKSTRTAYMELSSLRSKDTAVYYCARGNSRSDAFDIWGQGTMVTVSSGGGGSGGGGSGGGASSYELTHPPSVSVSPGQTASITCSGDKLGDKFVSWYHQKPGQSPVLVIYQDSKRPSGIPERFSGSNSGNTATLTISGTRAMDEADYYCQAWDSSTVVFGGGTKLTVLRTAAASAHHHHHHKLDYKDHDGDYKDHDIDYKDDDDK

SEQ ID NO: 179 - protein, 279 aa, artificial sequence
  scFv sequence G4_22
QVQLVESGGGLVQPGGSLRLSCAASGFTFSTYAMSWVRQAPGKGLEWVSTVSGSGGTTYYADSVKGRFTISRDNSKNTLYLQMNSLRAEDTAVYYCAKDSTAVTDWFDPWGRGTLVTVSSGGGGSGGGGSGGGASDIQMTQSPSSLSASVGDRVTITCQASQDISNYLNWYQQKPGKAPKLLIYAASSLQSGVPSRFSVSGSGTDFTLTISNLQPEDFATYYCQQSYSIPWTFGQGTKVEIKRTAAASAHHHHHHKLDYKDHDGDYKDHDIDYKDDDDK

SEQ ID NO: 180 - protein, 279 aa, artificial sequence
  scFv sequence G4_23
EVQLVESGGGVVQPGRSLRLSCAASGFTFSSYGMHWVRQAPGKGLEWVAVIWYDGSNKYYADSVKGRFTISRDNSKNTLYLQMNSLRAEDTAVYYCARGEVAALYYFDYWGQGTLVTVSSGGGGSGGGGSGGGASDIQMTQSPSSLSASVGDRVTITCRASQGISNSLAWYQQKPGKAPKLLLYAASRLESGVPSRFSGSGSGTDYTLTISSLQPEDFATYYCQQYYSTPRTFGGGTKLEIKRTAAASAHHHHHHKLDYKDHDGDYKDHDIDYKDDDDK

SEQ ID NO: 181 - protein, 287 aa, artificial sequence
  scFv sequence G4_24
QVQLQQSGPGLVKPSQTLSLTCAISGASVSSNSVAWNWIRQSPSRGLEWLGRTYYRSRWYNDYALSVKSRIIINPDTSKNQFSLQLNSVTPEDTAVYYCARDWSSTRSFDYWGRGTLVTVSSGGGGSGGGGSGGGASDIVMTQSPDSLAVSLGERATINCKSSQSVLYSSNNKNYLAWYQQKPGQPPKLLISWASTRESGVPDRFSGSGSGTDFTLTINSLQSEDVAIYYCQQYYSTPPTFGQGTKLEIKRTAAASAHHHHHHKLDYKDHDGDYKDHDIDYKDDDDK

SEQ ID NO: 182 - protein, 283 aa, artificial sequence
  scFv sequence G4_25
EVQLVESGAEVKKPGSSVKVSCKASGGTFSSYAISWVRQAPGQGLEWMGGIIPIFGTANYAQKFQGRVTITADKSTSTAYMELSSLRSEDTAVYYCARSLRDGYNYIGSLGYWGQGTLVTVSSGGGGSGGGGSGGGASQSALTQPRSVSGSPGQSVTISCTGTSSDVGGYNYVSWYQQHPGKAPKLMIYEVSNRPSGVSNRFSGSKSGNTASLTISGLQAEDEADYYCSSYGSGSVFGTGTKLTVLRTAAASAHHHHHHKLDYKDHDGDYKDHDIDYKDDDDK

SEQ ID NO: 183 - protein, 280 aa, artificial sequence
  scFv sequence G4_26
QVQLVQSGAEVKKPGSSVKVSCKASGGTFSSYAISWVRQAPGQGLEWMGGIIPIFGTANYAQKFQGRVTITADESTSTAYMELSSLRSEDTAVYYCASSRGSGWFPLGYWGQGTLVTVSSGGGGSGGGGSGGGASQSGLTQPASVSGSPGQSITISCTGTSSDVGSYNLVSWYQQHPGKAPKLMIYEVSKRPSGVSNRFSGSKSGNTASLTISGLQAEDEADYYCSSFGSGSIFGTGTKLTVLRTAAASAHHHHHHKLDYKDHDGDYKDHDIDYKDDDDK

SEQ ID NO: 184 - protein, 282 aa, artificial sequence
  scFv sequence G4_27
QVQLVQSGAEVKKPGESLKISCKSSGYSFTSYWIGWVRQMPGKGLEWMGIIYPGDSDTRYSPSFQGQVTFSADESISTAYLQWSSLKASDTAMYYCARHGAYGDYPDTFDIWGQGTLVTVSSGGGGSGGGGSGGGASSYELTQDPAVSVALGQTVSITCQGDSLRNFYANWYQQKPGQAPVLVIYGKNNRPSGIPDRFSGSSSGNTASLTITGAQAEDEADYYCNSRDSSGNHLVFGGGTQLTVLRTAAASAHHHHHHKLDYKDHDGDYKDHDIDYKDDDDK

SEQ ID NO: 185 - protein, 283 aa, artificial sequence
  scFv sequence G4_28
QVQLVESGGGLVQPGGSLRLSCAASGFTFDDYAMHWVRQAPGKGLEWVSGISAGGGSTNYAGSVKGRFTVSRDTSKNTLYLQMNSLRAEDTAVYYCVKSYVDTAMRYYYYYMDVWGQGTMVTVSSGGGGSGGGGSGGGASSYELTQDPAVSVALGQTVTITCQGDSLRNYYASWYRQKPGQTPVLVVYGKNNRPSGIPDRFSVSASGNTASLTITGAQAEDEGDYYCNSRDSSGVVFGGGTKVTVLRTAAASAHHHHHHKLDYKDHDGDYKDHDIDYKDDDDK

SEQ ID NO: 186 - protein, 13 aa, artificial sequence
  Linker
GGGGSGGGGSGGG

SEQ ID NO: 187 - DNA, 348 bp, artificial sequence
  Nucleotide VH sequence G4_1
gaggtgcagctgttggagtctgggggaggcgtggtccagcctgggaggcccctgagactctcctgtgcagcgtctggattcaccttcagtagctatagcatgaactgggtccgccaggctccagggaaggggctggagtgggtctcatccattagtagtagtagtagttacatatactacgcagactcagtgaagggccgattcaccatctccagagacaattccaagaacacgctgtatctgcaaatgaacagcctgagagccgaggacacggccgtatattactgtgcgaaaggacactggtacttcgatctctggggccgtggcaccctggtcaccgtctcgagt

SEQ ID NO: 188 - DNA, 360 bp, artificial sequence
  Nucleotide VH sequence G4_2
cagatgcagctggtgcagtctggggctgaggtgaagaagcctggggctacagtgaaaatctcctgcaaggtttctggataccctttcaccgactactatatccactgggtgcaacaggcccctggaaaagggcttgagtggatgggacttgttgatcctgaggatgggcaaagtagatccgcggagaggttccagggcagagtcaccataaccgcggacacgtctacagacacagcctacatggagctgagcagcctgagatctgaggacacggccgtgtattactgtgcaacattcccagtggctggattctacggtatggacgtctggggccagggaaccctggtcaccgtctcgagt

SEQ ID NO: 189 - DNA, 348 bp, artificial sequence
  Nucleotide VH sequence G4_3
gaggtgcagctggtggagtccgggggaggcttggtccagccgggggggtccctgagactctcctgtgcagcctctggattcaccttcagtagctatagcatgaactgggtccgccaggctccagggaaggggctggagtgggtctcatccattagtagtagtagtagttacatatactacgcagactccgtgaagggccggttcaccatctccagagacaattccaagaacacgctgtatctgcaaatgaacagcctgagagccgaggacacggccgtgtattactgtgcgagaggagggtggctatatgactactggggccaaggaaccctggtcaccgtctcgagt

SEQ ID NO: 190 - DNA, 357 bp, artificial sequence
  Nucleotide VH sequence G4_4
caggtgcagctggtggagtctgggggaggcttggtacagcctggggggtccctgagactctcctgtgcagcctctggattcacctttagcagctatgccatgagctgggtccgccaggctccagggaaggggctggagtgggtctcagctattagtggtagtggtggtagcacatactacgcagactccgtgaagggccggttcaccatctccagagacaattccaaaaacaccctgtatctgcaaatgagcagcctgagagtcgaagacacggccgtatattattgtgcgaaatcgtcggtgggctggtggtcttttgactactggggccaagggacaatggtcaccgtctcgagt

SEQ ID NO: 191 - DNA, 360 bp, artificial sequence
  Nucleotide VH sequence G4_5
gaagtgcagctggtgcagtctggggctgaggtgaagaagcctgggtcctcggtgaaggtctcctgcaaggcttctggttacacctttaccagctacggtatcagctgggtgcgacaggcccctggacaagggcttgagtggatgggatggatcggcgcttacaatggtaacacaaactatgcacagaagctccagggcagagtcaccatgagcacagacacatccacgagcacagcctacatggagctgaggagcccgagatctgacgacacggccgtgtattactgtgcgagaggcgggacggggggtgaccacgtctttgcctactgggggcaagggaccacggtcaccgtctcgagt

SEQ ID NO: 192 - DNA, 360 bp, artificial sequence
  Nucleotide VH sequence G4_6
gaggtgcagctggtggagtctgggggaggcttggtacagcctggggggcccctgagactctcctgtgcagcctctggattcacctttagcagctatgccatgaactgggtccgccaggctccagggaaggggctggagtgggtctcagctattagtggtagtggtggtagcacatactacgcagactccgtgaagggccggttcaccatctccagagacaattccaagaacacgctgtatctgcaaatgaacagcctgagagccgaggacacggccgtatattactgtgcgaaagccgactacggggtggtctactactttgactactggggccaagggacaatggtcaccgtctcgagt

SEQ ID NO: 193 - DNA, 357 bp, artificial sequence
  Nucleotide VH sequence G4_7
gaggtgcagctggtggagtctgggggaggctgggtccagtctggggggtccctgagaccctcctgtgcagcctctggattcacctttagtcactattggatgagttgggtccgccaggctccagggaaggggctggagtgggtggccaacataaagcaagatggaagtatcatatactatgcagactctgtgaagggccgattcaccatctccagggacaacgccaagaactcagtgtatctgcaaatgaacagcctgagagccgaggacacggctgtgtattactgtgcgagaattgggtatagcagctcgtcttttgactactggggccgtggcaccctggtcaccgtctcgagt

SEQ ID NO: 194 - DNA, 366 bp, artificial sequence
  Nucleotide VH sequence G4_10
caggtgcagctggtggagtctgggggaggcgtggtccagcctgggaggcccctgagactctcctgtgcagcctctggattcaccttcagtagctatgctatgcactgggtccgccaggctccagggaaggggctggagtgggtctcagctattagtggtagtggtggtagcacatactacgcagactccgtgaagggccggttcaccatctccagagacaattccaagaacacgctgtatctgcaaatgaacagcctgagagccgaggacacggccgtatattactgtgcgaaagatggggccgtggatttttggcgaaacggtatggacgtctggggccgtggcaccctggtcaccgtctcgagt

SEQ ID NO: 195 - DNA, 351 bp, artificial sequence
  Nucleotide VH sequence G4_12
gaggtgcagctgttggagtctggaggaggcttggtccagcctggggggtccctgagactctcctgtgcagcctctgggttcaccgtcagtagcaactacatgagctgggtccgccaggctccagggaaggggctggagtgggtctcagttatttatagcggtggtagcacatactacgcagactccgtgaagggccgattcaccatctcccgacacaattccaagaacacgctgtatcttcaaatgaacagcctgagagctgaggacacggccgtgtattactgtgcgagagtagcgaacggtgactttcttgactactggggccgtggcaccctggtcaccgtctcgagt

SEQ ID NO: 196 - DNA, 351 bp, artificial sequence
  Nucleotide VH sequence G4_13
caggtgcagctggtggagtctggggctgaggtgaagaagcctggggggtccctgagactctcctgtgcagcctctggattcaccttcagtagctatagcatgaactgggtccgccaggctccagggaaggggctggagtgggtctcatccattagtggtactagtagttacatatactacgcagactctgtgaagggccgattcaccatctccagagacaacgccaagaactcactgtatctgcaaatgagcagcctgagagccgaggacacggctgtttattactgtgcgagaggagggctcgggatggtcgacccctggggccagggaaccctggtcaccgtctcgagt

SEQ ID NO: 197 - DNA, 351 bp, artificial sequence
  Nucleotide VH sequence G4_14
gaagtgcagctggtgcagtccggagcagaggtgaaaaagcccggggagtctctgaggatctcctgtaagggttctggatacagctttaccagctactggatcagctgggtgcgccagatgcccgggaaaggcctggagtggatggggaggattgatcctagtgactcttataccaactacagcccgtccttcccaggccacgtcaccatctcagctgacaagtccatcagcactgcctacctgcagtggagcagcctgaaggcctcggacaccgccatgtattactgtgcggcggatacagctcacggtatggacgtctggggccgtggcaccctggtcaccgtctcgagt

SEQ ID NO: 198 - DNA, 366 bp, artificial sequence
  Nucleotide VH sequence G4_15
gaagtgcagctggtgcagtctgaggctgaggtgaagaagcctggggcctcagtgaaggtttcctgcaaggcctctggatacaccttcaccaggcattatatgcactgggtgcgacaggcccccggacaagggcttgagtggatgggactaatcaaccctagtggtagtagcacagtctacgcacagaagttccagggcagagtcaccttgaccagggacacgtccacgagcacagactacatggagctgagcagcctgagatctgaggacacggccgtctattattgtgcgagagataatagtcacctcgaccaggtttggtggttcgacccctggggccagggcaccctggtcaccgtctcgagt

SEQ ID NO: 199 - DNA, 357 bp, artificial sequence
  Nucleotide VH sequence G4_16
gaggtgcagctgttggagtctggagctgaggtgaagaagcctggggcctcagtgaaggtctcctgcaaggcttctggttacacctttaccagctatggtatcagctgggtgcgacaggcccctggacaagggcttgagtggatgggatggatcagcgcttacaatggtaacacaaactatgcacagaagctccagggcagagtcaccatgaccacagacacatccacgagcacagcctacatggagctgaggagcctgagatctgacgacacggccgtgtattactgtgcgagagactacggtgacttctacggtatggacgtctggggccaaggaaccctggtcaccgtctcgagt

SEQ ID NO: 200 - DNA, 354 bp, artificial sequence
  Nucleotide VH sequence G4_18
gaggtgcagctggtggagtctggggctgaggtgaagaagcctggggcctcagtgaaggtctcctgcaaggcttctggatacaccttcaccggctactatatgcactgggtgcgacaggcccctggacaagggcttgagtggatgggacggatcaaccctaacagtggtggcacaaactatgcacagaagtttcagggcagggtcaccatgaccagggacgcgtccatcagcacagcctacatggagctgagcaggctgagatctgacgacacggccgtgtattactgtgcgagagatcttgatctatcctcccttgactactggggccgtggcaccctggtcaccgtctcgagt

SEQ ID NO: 201 - DNA, 363 bp, artificial sequence
  Nucleotide VH sequence G4_19
gaagtgcagctggtgcagtctggggctgaggtgaagaagcctggggcctcagtgaaggtttcctgcaaggcatctggatacaccctcaccagctactatatgcactgggtgcgacaggcccctggacaagggcttgagtggatgggaataatcaaccctagtggtggtagcacaagctacgcacagaagttccagggcagagtcaccatgaccagggacacgtccacgagcacagtctacatggagctgagcagcctgagatctgaggacacggccgtgtattactgtgcgagagagcgtggatacagctatggtgacggtatggacgtctgggggcaagggaccacggtcaccgtctcgagt

SEQ ID NO: 202 - DNA, 357 bp, artificial sequence
  Nucleotide VH sequence G4_20
caggtgcagctggtggagtctggagctgaggtgaagaagcctggggcctcggtgaaggtctcctgcaaggcttctggaggcaccttcagcagctatgctatcagctgggtgcgacaggcccctggacaagggcttgagtggatgggagggatcatccctatctttggtacagcaaactacgcacagaagttccagggcagagtcacgattaccgtggacaaatccacgcgcacagcctacatggagctgagcagcctgagatctaaggacacggccgtgtattactgtgcgagggggaatagcagaagtgatgcttttgatatctggggccaagggacaatggtcaccgtctcgagt

SEQ ID NO: 203 - DNA, 360 bp, artificial sequence
  Nucleotide VH sequence G4_22
caggtgcagttggtggagtctgggggaggcttggtacagcctggggggtccctgagactctcctgtgcagcctctggattcacctttagcacctatgccatgagctgggtccgccaggctccagggaaggggctggagtgggtctcaactgttagtggtagtggtggtaccacatactacgcagactccgtgaagggccggttcaccatctccagagacaattccaagaacacgctgtatctgcaaatgaacagcctgagagccgaagacacggccgtatattactgtgcgaaagattcaacggcggtgactgactggttcgacccctggggccgtggcaccctggtcaccgtctcgagt

SEQ ID NO: 204 - DNA, 360 bp, artificial sequence
  Nucleotide VH sequence G4_23
gaggtgcagctggtggagtctgggggaggcgtggtccagcctgggaggtccctgagactctcctgtgcagcgtctggattcaccttcagtagctatggcatgcactgggtccgccaggctccaggcaaggggctggagtgggtggcagttatatggtatgatggaagtaataaatactatgcagactccgtgaagggccgattcaccatctccagagacaattccaagaacacgctgtatctgcaaatgaacagcctgagagccgaggacacggctgtgtattactgtgcgagaggggaagtggctgccttgtactactttgactactggggccagggaaccctggtcaccgtctcgagt

SEQ ID NO: 205 - DNA, 366 bp, artificial sequence
  Nucleotide VH sequence G4_24
caggtacagctgcagcagtcaggtccaggactggtgaagccctcgcagaccctctcactcacctgtgccatctccggggccagtgtctctagcaacagtgttgcttggaactggatcaggcagtccccatcgagaggccttgagtggctggggaggacatactacaggtccaggtggtataatgattatgcattatctgtgaaaagtcgaataatcatcaacccagacacatccaagaaccagttctccctgcagctgaactctgtgacccccgaggacacggctgtgtattactgtgcaagagattggagcagcacccgatcctttgactactggggccgtggcaccctggtcaccgtctcgagt

SEQ ID NO: 206 - DNA, 369 bp, artificial sequence
  Nucleotide VH sequence G4_25
gaggtgcagctggtggagtctggggctgaggtgaagaagcctgggtcctcggtgaaggtctcctgcaaggcttctggaggcaccttcagcagctatgctatcagctgggtgcgacaggcccctggacaagggcttgagtggatgggagggatcatccctatctttggtacagcaaactacgcacagaagttccagggcagagtcacgattaccgcggacaaatccacgagcacagcctacatggagctgagcagcctgagatctgaggacacggccgtgtattactgtgcgagatctcttagagatggctacaattacatcggaagtttaggctactggggccagggcaccctggtcaccgtctcgagt

SEQ ID NO: 207 - DNA, 360 bp, artificial sequence
  Nucleotide VH sequence G4_26
caggtccagcttgtgcagtctggggctgaggtgaagaagcctggatcctcggtgaaggtctcctgcaaggcttctggaggcaccttcagcagctatgctatcagctgggtgcgacaggcccctggacaagggcttgagtggatgggagggatcatccctatctttggtacagcaaactacgcacagaagttccagggcagagtcacgattaccgcggacgaatccacgagcacagcttacatggagctgagcagcctgagatctgaagacacggctgtgtattactgtgcgagctcccggggcagtggctggtttcctttgggttactggggccaaggaaccctggtcaccgtctcgagt

SEQ ID NO: 208 - DNA, 366 bp, artificial sequence
  Nucleotide VH sequence G4_27
caggtccagctggtacagtctggagcagaggtgaaaaagcccggggagtctctgaagatctcctgtaagagttctggatacagctttaccagctactggatcggctgggtgcgccagatgcccgggaaaggcctggagtggatggggatcatctatcctggtgactctgataccagatacagcccgtccttccaaggccaggtcaccttctcagccgacgagtccatcagtaccgcctacctgcagtggagcagcctgaaggcctcggacaccgccatgtattactgtgcgagacatggcgcctacggtgactacccggatacttttgatatctggggccagggcaccctggtcaccgtctcgagt

SEQ ID NO: 209 - DNA, 375 bp, artificial sequence
  Nucleotide VH sequence G4_28
caggtgcagctggtggagtctgggggaggcttggtacagcctggggggtccctgagactctcctgtgcagcctctggattcacctttgatgattatgccatgcactgggtccggcaagctccagggaaggggctggagtgggtctcaggtattagtgctggtggtggtagcacaaactacgcaggctccgtgaagggccggttcaccgtctccagggacacgtccaagaacacactttatctgcaaatgaacagcctgagagccgaggacacggccgtgtattactgtgtgaagtcctacgtggatacagctatgcgctactactactactacatggacgtctggggccaagggacaatggtcaccgtctcgagt

SEQ ID NO: 210 - DNA, 321 bp, artificial sequence
  Nucleotide VL sequence G4_1
gacatccagatgacccagtctccatcctccctgtctgcatctgtaggagacagagtcaccatcacttgccaggcgagtcaggacattagcaactatttaaattggtatcagcagaaaccagggaaagcccctaagctcctgatctacgatgcatccaatttggaaacaggggtcccatcaaggttcagtggaagtggatctgggacagatttcactctcaccatcagcagtctgcaacctgaagattttgcaacttactactgtcaacagagttacagtacccccgtcactttcggccctgggaccaaggtggaaatcaaa

SEQ ID NO: 211 - DNA, 321 bp, artificial sequence
  Nucleotide VL sequence G4_2
gacatccagatgacccagtctccatcctccctgtctgcatctgtaggagacagagtcaccatcacttgccaggcgagtcaggacattagcaactatttaaattggtatcagcagaaaccagggaaagcccctaagctcctgatctatgctgcatccagtttgcaaagtggggtcccatcaaggttcagtggcagtggatctgggacagatttcactctcaccatcagcggcctgcagcctgaagattttgcaacttactactgtctagaagattacaactacctgtggacgttcggccaagggaccaagctggagatcaaa

SEQ ID NO: 212 - DNA, 321 bp, artificial sequence
  Nucleotide VL sequence G4_3
gacatccagatgacccagtctccatcctccctgtctgcatctgtaggagacagagtcaccatcacttgccaggcgagtcaggacattagcaactatttaaattggtatcagcagaaaccagggaaagcccctaagctcctgatctacgatgcatccaatttggaaacaggggtcccatcaaggttcagtggaagtgggtctgggacagatttcactctcaccatcagcagtctgcaacctgaagattttgcaacttacttctgtcaacagagttacagtaccccccagacgttcggccaagggaccaaagtggatatcaaa

SEQ ID NO: 213 - DNA, 339 bp, artificial sequence
  Nucleotide VL sequence G4_4
gatattgtgatgacccagtctccagactccctggctgtgtctctgggcgagagggccaccatcaactgcaagtccagccagagtgttttgtccagctccaacaataacaactacttagcttggtaccaacagagaccaggacagcctcctaagctgctcttttactgggcatctacccgggaatcgggggtccctgaccgattcagtggcagcgggtctggaacatctttcactctcaccatcaccagcctgcaggctgaagatgtggcggtttattactgtcagcaatattattccactcctctcactttcggcggagggaccaagctggagatcaaa

SEQ ID NO: 214 - DNA, 321 bp, artificial sequence
  Nucleotide VL sequence G4_5
gacatccagatgacccagtctccatcctccctgtctgcatctgtaggagacagagtcaccatcacttgccgggcaagtcagagcattagcagctatttaaattggtatcagcagaaaccagggaaagcccctaagctcctgatctatgctgcatccagtttgcaaagtggggtcccatcaaggttcagcggcagtggatctgggacagatttcactctcactatcagcagcctgcagcctgaagattttgcaacttactactgtcaacagagttacagtaccccctacacttttggccaggggaccaaggtggaaatcaaa

SEQ ID NO: 215 - DNA, 321 bp, artificial sequence
  Nucleotide VL sequence G4_6
gacatccagatgacccagtctccatcctccctgtctgcatctgtaggagacagagtcaccatcacttgccgggcaagtcagagcattagcacctatttaaattggtatcagcagaaaccagggaaagcccctaagctcctgatctatgctgcatccagtttgcagagtggggtcccatcaaggttcagtggcagtggatctgggacagatttcactctcaccatcagcagtccgcaacctgaagattttgcaacttactactgtcaacagagttacagtaccccgtacacttttggccaggggaccaaggtggaaatcaaa

SEQ ID NO: 216 - DNA, 336 bp, artificial sequence
  Nucleotide VL sequence G4_7
gatattgtgatgacgcagtctccactctccctgcccgtcacccctggagagccggcctccatctcctgcaggtccagtcagagcctcctgcatagtaatagattcaactatttggattggtacctgcagaagccagggcagtctccacagctcctgatctatttgggttctaatcgggcctccggggtccctgacaggttcagtggcagtggatctggcacagattttacactgaaaatcagcagagtggaggctgaggatgttggggtttattactgcatgcaaggtctacaaactccgtacacttttggccaggggaccaaagtggatatcaaa

SEQ ID NO: 217 - DNA, 336 bp, artificial sequence
  Nucleotide VL sequence G4_10
gatattgtgatgacgcagcctccactctccctgcccgtcacccttggacatccggcctccatctcctgcaagtctagtcaaagcctcgaatatagtgatggaaacacctacttgaattggtttcagcagaggccaggccaatctccaaggcgcctcatttataaggtttctaaccgggactctggggcccccgacagattcagcgggagtgggtcaggcactgatttcacactggaaatcagcagggtggaggctgaggatgttggagtttattactgtatgcaaggtacactctggcctcccacgttcggccaagggaccaaagtggatatcaaa

SEQ ID NO: 218 - DNA, 324 bp, artificial sequence
  Nucleotide VL sequence G4_12
cagtctgtgctgactcagcctgcctccgtgtctgggtctcctggacagtcgatcaccatctcctgcactggaaccagcagtgacgttggtggttataactttgtctcctggtaccaacaacacccaggcaaagcccccaaactcatgatttatgaggtcactaatcggccctcaggggtccctgatcggttctctggctccaagtctggcaacacggcctccctgaccatctctgggctccaggctgaggacgaggctgattattactgcagctcacatgcaagccccagggtcttcggaactgggaccaaggtcaccgtccta

SEQ ID NO: 219 - DNA, 333 bp, artificial sequence
  Nucleotide VL sequence G4_13
aattttatgctgactcagccccactctgtgtcggagtctccggggaagacggtaaccatctcctgcacccgcagcagtggcagcattgccagcaactatgtgcagtggtaccagcagcgcccgggcagttcccccagcactgtgatctatgaggataaccaaagaccctcaggggtccctgatcggttctctggctccatcgacagctcctccaactctgcctccctcaccatctctggactgaggactgaggacgaggctgactactactgtcagtcttatgatagcagcatttatgtggtattcggcggagggaccaagctgaccgtccta

SEQ ID NO: 220 - DNA, 333 bp, artificial sequence
  Nucleotide VL sequence G4_14
aattttatgctgactcagccccactctgtgtcggagtctccggggaagacggtaaccatatcctgcacccgcagccgtggcagcattgccggcaactatgtgcactggtaccagcagcgcccagggcgtgcccccaccactgtgatctatcgggataaggaaagaccctctggggtccctgatcgaatctctggctccatcgacagctcctccaactctgcctccctcaccatctctggactgaagactgaggacgaggctgattactattgtcagtcttatgatagcagcacccatgtggtattcggcggagggaccaagctgaccgtccta

SEQ ID NO: 221 - DNA, 324 bp, artificial sequence
  Nucleotide VL sequence G4_15
cagtctgcgctgactcagcctgcctccgtgtctgggtctcctggacagtcgatcaccatctcctgcactggaaccagcagtgacgttggtggttataactatgtctcctggtaccaacaacacccaggcaaagcccccaaactcatgatttatgacgtcagtaatcggccctcaggggtttctaatcgcttctctggctccaagtctggcaacacggcctccctgaccatctctgggctccaggctgaggacgaggctgattattactgcagctcgtatggaagcggcagcgtcttcggaactgggaccaagctgaccgtccta

SEQ ID NO: 222 - DNA, 330 bp, artificial sequence
  Nucleotide VL sequence G4_16
cagtctgtgctgactcagcctccctccgcgtccgggtctcctggacagtcagtcaccttctcctgcactggaaccagcagtgacattggtgcttttaactctgtctcttggtaccaacagcacccaggcaaagcccccaaactcctaatttatgagatcactaagcggccctcaggggtccctgatcgcttctctggctccaagtctggcaacacggcctccctgaccatctctgtgctccaggctgaagatgaggctgattattactgcacctcatatgcaggcagcaacactttgatcttcggcggagggaccaaggtcaccgtccta

SEQ ID NO: 223 - DNA, 324 bp, artificial sequence
  Nucleotide VL sequence G4_18
tcctatgagctgacacagccaccctcggtgacagagtccccaggacagacggccaggatcacctgctctggagatgcattggcaaagcaatatgcttattggtaccagcagaagccaggccaggcccctgtgttggtgatatatagagacagtgagaggccttcagagatccctgagcgattctctggctccagctcagggacaacagtcacgttgaccatcagtggagtccaggcagaagacgaggctgactattactgtcaatcagcagacagcagtggtacttatacagtatttggcggagggaccaagctgaccgtccta

SEQ ID NO: 224 - DNA, 333 bp, artificial sequence
  Nucleotide VL sequence G4_19
aattttatgctgactcagccccactctgtgtcggagtctccggggaagacggtcaccatctcctgcacccgcagcagtggcagcattgccagcaactatgtacagtggtaccagcagcgcccgggcagtccccccatcactttgatatatgatgatgaccaaagaccctctggggtccctcatcggttctctggctccatcgacacctcatccaaccctgcctccctcaccatctctggactgaagactgaggacgaggctgactactactgtcagtcttatgatagcagcaatcatgtggtattcggcggagggaccaagctgaccgtccta

SEQ ID NO: 225 - DNA, 318 bp, artificial sequence
  Nucleotide VL sequence G4_20
tcctatgagctgactcatccaccctcagtgtccgtgtccccaggacagacagccagcatcacctgctctggagataaattgggggataagtttgtttcctggtatcaccaaaagccaggccagtcccctgtgctggtcatctatcaagatagcaagcggccctcagggatccctgagcgcttctcaggctccaattctgggaacacagccactctgaccatcagcgggacccgggctatggatgaggctgactattactgtcaggcgtgggacagcagcactgtggtattcggcggagggaccaagctgaccgtccta

SEQ ID NO: 226 - DNA, 321 bp, artificial sequence
  Nucleotide VL sequence G4_22
gacatccagatgacccagtctccatcctccctgtctgcatctgtaggagacagagtcaccatcacttgccaggcgagtcaggacattagcaactatttaaattggtatcagcagaaaccagggaaagcccctaagctcctgatctatgctgcatccagtctgcaaagtggggtcccatcaaggttcagcgtcagtggatctgggacagatttcactctcaccatcagcaacctgcagcctgaagattttgcaacttattactgtcaacagagttacagtatcccgtggacgttcggccaagggaccaaggtggagatcaaa

SEQ ID NO: 227 - DNA, 321 bp, artificial sequence
  Nucleotide VL sequence G4_23
gacatccagatgacccagtctccatcctccctgtctgcatctgtaggagacagagtcaccatcacttgccgggcgagtcagggcattagcaattctttagcctggtatcagcagaaaccagggaaagcccctaagctcctgctctatgctgcgtccagattggaaagtggggtcccatccaggtttagtggcagtggatctgggacggattacaccctcaccatcagcagcctgcagcctgaagattttgcaacttattactgtcaacagtattatagtacccctcgcactttcggcggagggaccaagctggagatcaaa

SEQ ID NO: 228 - DNA, 339 bp, artificial sequence
  Nucleotide VL sequence G4_24
gatattgtgatgacccagtctccagactccctggctgtgtctctgggcgagagggccaccatcaactgcaagtccagccagagtgttttatacagctccaacaataagaactacttagcttggtaccagcagaaaccaggacagcctcctaagttgttgatttcctgggcttctacccgggaatctggggtccctgaccgattcagtggcagcgggtctgggacagatttcactctcaccatcaacagcctacagtctgaagatgtggcaatttattactgtcagcaatattattctacccctccgacgttcggccaggggaccaagctggagatcaaa

SEQ ID NO: 229 - DNA, 324 bp, artificial sequence
  Nucleotide VL sequence G4_25
cagtctgcgctgactcagcctcgctcagtgtccgggtctcctggacagtcagtcaccatctcctgcactggaaccagcagtgatgttggtggttataactatgtctcctggtaccaacagcacccaggcaaagcccccaaactcatgatttatgaggtcagtaatcggccctcaggggtttctaatcgcttctctggctccaagtctggcaacacggcctccctgaccatctctgggctccaggctgaggacgaggctgattattactgcagctcgtatggaagcggcagcgtcttcggaactgggaccaagctgaccgtccta

SEQ ID NO: 230 - DNA, 324 bp, artificial sequence
  Nucleotide VL sequence G4_26
cagtctgggctgactcagcctgcctccgtgtctgggtctcctggacagtcgatcaccatctcctgcactggaaccagcagtgatgttgggagttataaccttgtctcctggtaccaacagcacccaggcaaagcccccaaactcatgatttatgaggtcagtaagcggccctcaggggtttctaatcgcttctctggctccaagtctggcaacacggcctccctgaccatctctgggctccaggctgaggacgaggctgattattactgcagctcgtttggaagcggcagcatcttcggaactgggaccaagctgaccgtccta

SEQ ID NO: 231 - DNA, 324 bp, artificial sequence
  Nucleotide VL sequence G4_27
tcctatgagctgactcaggacccagctgtgtctgtggccctgggacagacagtcagtatcacatgccaaggagacagcctcagaaacttttatgcaaactggtaccagcaaaagccaggacaggcccctgtacttgtcatctatggtaaaaacaaccggccctcagggatcccagaccgattctctggctccagctcaggaaacacagcttccttgaccatcactggggctcaggcggaagatgaggctgactattactgtaactcccgggacagcagtggtaaccatctggtattcggcggagggacccagctcaccgtccta

SEQ ID NO: 232 - DNA, 318 bp, artificial sequence
  Nucleotide VL sequence G4_28
tcctatgagctgactcaggaccctgctgtgtctgtggccttgggacagacagtcacgatcacatgccaaggagacagcctcagaaactattatgcaagctggtaccggcagaagccaggacagacccctgtacttgtcgtctatggtaaaaacaaccggccctcagggatcccagaccgattctctgtctccgcctcaggtaacacagcttccttgaccatcactggggctcaggcggaagatgagggtgactattactgtaactcccgggacagcagtggtgtggttttcggcggagggaccaaggtcaccgtccta

SEQ ID NO: 233 - protein, 662 aa, artificial sequence
  G4_1 IgG1 antibody sequence?
ASDIQMTQSPSSLSASVGDRVTITCQASQDISNYLNWYQQKPGKAPKLLIYDASNLETGVPSRFSGSGSGTDFTLTISSLQPEDFATYYCQQSYSTPVTFGPGTKVEIKRTAAAPSVFIFPPSDEQLKSGTASVVCLLNNFYPREAKVQWKVDNALQSGNSQESVTEQDSKDSTYSLSSTLTLSKADYEKHKLYACEVTHQGLSSPVTKSFNRGECEVQLLESGGGVVQPGRPLRLSCAASGFTFSSYSMNWVRQAPGKGLEWVSSISSSSSYIYYADSVKGRFTISRDNSKNTLYLQMNSLRAEDTAVYYCAKGHWYFDLWGRGTLVTVSSASTKGPSVFPLAPSSKSTSGGTAALGCLVKDYFPEPVTVSWNSGALTSGVHTFPAVLQSSGLYSLSSVVTVPSSSLGTQTYICNVNHKPSNTKVDKKVEPKSCDKTHTCPPCPAPELLGGPSVFLFPPKPKDTLMISRTPEVTCVVVDVSHEDPEVKFNWYVDGVEVHNAKTKPREEQYNSTYRVVSVLTVLHQDWLNGKEYKCKVSNKALPAPIEKTISKAKGQPREPQVYTLPPSRDELTKNQVSLTCLVKGFYPSDIAVEWESNGQPENNYKTTPPVLDSDGSFFLYSKLTVDKSRWQQGNVFSCSVMHEALHNHYTQKSLSLSPGK

SEQ ID NO: 234 - protein, 666 aa, artificial sequence
  G4_2 IgG1 antibody sequence
ASDIQMTQSPSSLSASVGDRVTITCQASQDISNYLNWYQQKPGKAPKLLIYAASSLQSGVPSRFSGSGSGTDFTLTISGLQPEDFATYYCLEDYNYLWTFGQGTKLEIKRTAAAPSVFIFPPSDEQLKSGTASVVCLLNNFYPREAKVQWKVDNALQSGNSQESVTEQDSKDSTYSLSSTLTLSKADYEKHKLYACEVTHQGLSSPVTKSFNRGECQMQLVQSGAEVKKPGATVKISCKVSGYPFTDYYIHWVQQAPGKGLEWMGLVDPEDGQSRSAERFQGRVTITADTSTDTAYMELSSLRSEDTAVYYCATFPVAGFYGMDVWGQGTLVTVSSASTKGPSVFPLAPSSKSTSGGTAALGCLVKDYFPEPVTVSWNSGALTSGVHTFPAVLQSSGLYSLSSVVTVPSSSLGTQTYICNVNHKPSNTKVDKKVEPKSCDKTHTCPPCPAPELLGGPSVFLFPPKPKDTLMISRTPEVTCVVVDVSHEDPEVKFNWYVDGVEVHNAKTKPREEQYNSTYRVVSVLTVLHQDWLNGKEYKCKVSNKALPAPIEKTISKAKGQPREPQVYTLPPSRDELTKNQVSLTCLVKGFYPSDIAVEWESNGQPENNYKTTPPVLDSDGSFFLYSKLTVDKSRWQQGNVFSCSVMHEALHNHYTQKSLSLSPGK

SEQ ID NO: 235 - protein, 662 aa, artificial sequence
  G4_3 IgG1 antibody sequence
ASDIQMTQSPSSLSASVGDRVTITCQASQDISNYLNWYQQKPGKAPKLLIYDASNLETGVPSRFSGSGSGTDFTLTISSLQPEDFATYFCQQSYSTPQTFGQGTKVDIKRTAAAPSVFIFPPSDEQLKSGTASVVCLLNNFYPREAKVQWKVDNALQSGNSQESVTEQDSKDSTYSLSSTLTLSKADYEKHKLYACEVTHQGLSSPVTKSFNRGECEVQLVESGGGLVQPGGSLRLSCAASGFTFSSYSMNWVRQAPGKGLEWVSSISSSSSYIYYADSVKGRFTISRDNSKNTLYLQMNSLRAEDTAVYYCARGGWLYDYWGQGTLVTVSSASTKGPSVFPLAPSSKSTSGGTAALGCLVKDYFPEPVTVSWNSGALTSGVHTFPAVLQSSGLYSLSSVVTVPSSSLGTQTYICNVNHKPSNTKVDKKVEPKSCDKTHTCPPCPAPELLGGPSVFLFPPKPKDTLMISRTPEVTCVVVDVSHEDPEVKFNWYVDGVEVHNAKTKPREEQYNSTYRVVSVLTVLHQDWLNGKEYKCKVSNKALPAPIEKTISKAKGQPREPQVYTLPPSRDELTKNQVSLTCLVKGFYPSDIAVEWESNGQPENNYKTTPPVLDSDGSFFLYSKLTVDKSRWQQGNVFSCSVMHEALHNHYTQKSLSLSPGK

SEQ ID NO: 236 - protein, 671 aa, artificial sequence
  G4_4 IgG1 antibody sequence
ASDIVMTQSPDSLAVSLGERATINCKSSQSVLSSSNNNNYLAWYQQRPGQPPKLLFYWASTRESGVPDRFSGSGSGTSFTLTITSLQAEDVAVYYCQQYYSTPLTFGGGTKLEIKRTAAAPSVFIFPPSDEQLKSGTASVVCLLNNFYPREAKVQWKVDNALQSGNSQESVTEQDSKDSTYSLSSTLTLSKADYEKHKLYACEVTHQGLSSPVTKSFNRGECQVQLVESGGGLVQPGGSLRLSCAASGFTFSSYAMSWVRQAPGKGLEWVSAISGSGGSTYYADSVKGRFTISRDNSKNTLYLQMSSLRVEDTAVYYCAKSSVGWWSFDYWGQGTMVTVSSASTKGPSVFPLAPSSKSTSGGTAALGCLVKDYFPEPVTVSWNSGALTSGVHTFPAVLQSSGLYSLSSVVTVPSSSLGTQTYICNVNHKPSNTKVDKKVEPKSCDKTHTCPPCPAPELLGGPSVFLFPPKPKDTLMISRTPEVTCVVVDVSHEDPEVKFNWYVDGVEVHNAKTKPREEQYNSTYRVVSVLTVLHQDWLNGKEYKCKVSNKALPAPIEKTISKAKGQPREPQVYTLPPSRDELTKNQVSLTCLVKGFYPSDIAVEWESNGQPENNYKTTPPVLDSDGSFFLYSKLTVDKSRWQQGNVFSCSVMHEALHNHYTQKSLSLSPGK

SEQ ID NO: 237 - protein, 666 aa, artificial sequence
  G4_5 IgG1 antibody sequence
ASDIQMTQSPSSLSASVGDRVTITCRASQSISSYLNWYQQKPGKAPKLLIYAASSLQSGVPSRFSGSGSGTDFTLTISSLQPEDFATYYCQQSYSTPYTFGQGTKVEIKRTAAAPSVFIFPPSDEQLKSGTASVVCLLNNFYPREAKVQWKVDNALQSGNSQESVTEQDSKDSTYSLSSTLTLSKADYEKHKLYACEVTHQGLSSPVTKSFNRGECEVQLVQSGAEVKKPGSSVKVSCKASGYTFTSYGISWVRQAPGQGLEWMGWIGAYNGNTNYAQKLQGRVTMSTDTSTSTAYMELRSPRSDDTAVYYCARGGTGGDHVFAYWGQGTTVTVSSASTKGPSVFPLAPSSKSTSGGTAALGCLVKDYFPEPVTVSWNSGALTSGVHTFPAVLQSSGLYSLSSVVTVPSSSLGTQTYICNVNHKPSNTKVDKKVEPKSCDKTHTCPPCPAPELLGGPSVFLFPPKPKDTLMISRTPEVTCVVVDVSHEDPEVKFNWYVDGVEVHNAKTKPREEQYNSTYRVVSVLTVLHQDWLNGKEYKCKVSNKALPAPIEKTISKAKGQPREPQVYTLPPSRDELTKNQVSLTCLVKGFYPSDIAVEWESNGQPENNYKTTPPVLDSDGSFFLYSKLTVDKSRWQQGNVFSCSVMHEALHNHYTQKSLSLSPGK

SEQ ID NO: 238 - protein, 666 aa, artificial sequence
  G4_6 IgG1 antibody sequence
ASDIQMTQSPSSLSASVGDRVTITCRASQSISTYLNWYQQKPGKAPKLLIYAASSLQSGVPSRFSGSGSGTDFTLTISSPQPEDFATYYCQQSYSTPYTFGQGTKVEIKRTAAAPSVFIFPPSDEQLKSGTASVVCLLNNFYPREAKVQWKVDNALQSGNSQESVTEQDSKDSTYSLSSTLTLSKADYEKHKLYACEVTHQGLSSPVTKSFNRGECEVQLVESGGGLVQPGGPLRLSCAASGFTFSSYAMNWVRQAPGKGLEWVSAISGSGGSTYYADSVKGRFTISRDNSKNTLYLQMNSLRAEDTAVYYCAKADYGVVYYFDYWGQGTMVTVSSASTKGPSVFPLAPSSKSTSGGTAALGCLVKDYFPEPVTVSWNSGALTSGVHTFPAVLQSSGLYSLSSVVTVPSSSLGTQTYICNVNHKPSNTKVDKKVEPKSCDKTHTCPPCPAPELLGGPSVFLFPPKPKDTLMISRTPEVTCVVVDVSHEDPEVKFNWYVDGVEVHNAKTKPREEQYNSTYRVVSVLTVLHQDWLNGKEYKCKVSNKALPAPIEKTISKAKGQPREPQVYTLPPSRDELTKNQVSLTCLVKGFYPSDIAVEWESNGQPENNYKTTPPVLDSDGSFFLYSKLTVDKSRWQQGNVFSCSVMHEALHNHYTQKSLSLSPGK

SEQ ID NO: 239 - protein, 670 aa, artificial sequence
  G4_7 IgG1 antibody sequence
ASDIVMTQSPLSLPVTPGEPASISCRSSQSLLHSNRFNYLDWYLQKPGQSPQLLIYLGSNRASGVPDRFSGSGSGTDFTLKISRVEAEDVGVYYCMQGLQTPYTFGQGTKVDIKRTAAAPSVFIFPPSDEQLKSGTASVVCLLNNFYPREAKVQWKVDNALQSGNSQESVTEQDSKDSTYSLSSTLTLSKADYEKHKLYACEVTHQGLSSPVTKSFNRGECEVQLVESGGGWVQSGGSLRPSCAASGFTFSHYWMSWVRQAPGKGLEWVANIKQDGSIIYYADSVKGRFTISRDNAKNSVYLQMNSLRAEDTAVYYCARIGYSSSSFDYWGRGTLVTVSSASTKGPSVFPLAPSSKSTSGGTAALGCLVKDYFPEPVTVSWNSGALTSGVHTFPAVLQSSGLYSLSSVVTVPSSSLGTQTYICNVNHKPSNTKVDKKVEPKSCDKTHTCPPCPAPELLGGPSVFLFPPKPKDTLMISRTPEVTCVVVDVSHEDPEVKFNWYVDGVEVHNAKTKPREEQYNSTYRVVSVLTVLHQDWLNGKEYKCKVSNKALPAPIEKTISKAKGQPREPQVYTLPPSRDELTKNQVSLTCLVKGFYPSDIAVEWESNGQPENNYKTTPPVLDSDGSFFLYSKLTVDKSRWQQGNVFSCSVMHEALHNHYTQKSLSLSPGK

SEQ ID NO: 240 - protein, 673 aa, artificial sequence
  G4_10 IgG1 antibody sequence
ASDIVMTQPPLSLPVTLGHPASISCKSSQSLEYSDGNTYLNWFQQRPGQSPRRLIYKVSNRDSGAPDRFSGSGSGTDFTLEISRVEAEDVGVYYCMQGTLWPPTFGQGTKVDIKRTAAAPSVFIFPPSDEQLKSGTASVVCLLNNFYPREAKVQWKVDNALQSGNSQESVTEQDSKDSTYSLSSTLTLSKADYEKHKLYACEVTHQGLSSPVTKSFNRGECQVQLVESGGGVVQPGRPLRLSCAASGFTFSSYAMHWVRQAPGKGLEWVSAISGSGGSTYYADSVKGRFTISRDNSKNTLYLQMNSLRAEDTAVYYCAKDGAVDFWRNGMDVWGRGTLVTVSSASTKGPSVFPLAPSSKSTSGGTAALGCLVKDYFPEPVTVSWNSGALTSGVHTFPAVLQSSGLYSLSSVVTVPSSSLGTQTYICNVNHKPSNTKVDKKVEPKSCDKTHTCPPCPAPELLGGPSVFLFPPKPKDTLMISRTPEVTCVVVDVSHEDPEVKFNWYVDGVEVHNAKTKPREEQYNSTYRVVSVLTVLHQDWLNGKEYKCKVSNKALPAPIEKTISKAKGQPREPQVYTLPPSRDELTKNQVSLTCLVKGFYPSDIAVEWESNGQPENNYKTTPPVLDSDGSFFLYSKLTVDKSRWQQGNVFSCSVMHEALHNHYTQKSLSLSPGK

SEQ ID NO: 241 - protein, 663 aa, artificial sequence
  G4_12 IgG1 antibody sequence
ASQSVLTQPASVSGSPGQSITISCTGTSSDVGGYNFVSWYQQHPGKAPKLMIYEVTNRPSGVPDRFSGSKSGNTASLTISGLQAEDEADYYCSSHASPRVFGTGTKVTVLGQPAAAPSVTLFPPSSEELQANKATLVCLISDFYPGAVTVAWKADSSPVKAGVETTTPSKQSNNKYAASSYLSLTPEQWKSHRSYSCQVTHEGSTVEKTVAPTECSEVQLLESGGGLVQPGGSLRLSCAASGFTVSSNYMSWVRQAPGKGLEWVSVIYSGGSTYYADSVKGRFTISRHNSKNTLYLQMNSLRAEDTAVYYCARVANGDFLDYWGRGTLVTVSSASTKGPSVFPLAPSSKSTSGGTAALGCLVKDYFPEPVTVSWNSGALTSGVHTFPAVLQSSGLYSLSSVVTVPSSSLGTQTYICNVNHKPSNTKVDKKVEPKSCDKTHTCPPCPAPELLGGPSVFLFPPKPKDTLMISRTPEVTCVVVDVSHEDPEVKFNWYVDGVEVHNAKTKPREEQYNSTYRVVSVLTVLHQDWLNGKEYKCKVSNKALPAPIEKTISKAKGQPREPQVYTLPPSRDELTKNQVSLTCLVKGFYPSDIAVEWESNGQPENNYKTTPPVLDSDGSFFLYSKLTVDKSRWQQGNVFSCSVMHEALHNHYTQKSLSLSPGK

SEQ ID NO: 242 - protein, 666 aa, artificial sequence
  G4_13 IgG1 antibody sequence
ASNFMLTQPHSVSESPGKTVTISCTRSSGSIASNYVQWYQQRPGSSPSTVIYEDNQRPSGVPDRFSGSIDSSSNSASLTISGLRTEDEADYYCQSYDSSIYVVFGGGTKLTVLGQPAAAPSVTLFPPSSEELQANKATLVCLISDFYPGAVTVAWKADSSPVKAGVETTTPSKQSNNKYAASSYLSLTPEQWKSHRSYSCQVTHEGSTVEKTVAPTECSQVQLVESGAEVKKPGGSLRLSCAASGFTFSSYSMNWVRQAPGKGLEWVSSISGTSSYIYYADSVKGRFTISRDNAKNSLYLQMSSLRAEDTAVYYCARGGLGMVDPWGQGTLVTVSSASTKGPSVFPLAPSSKSTSGGTAALGCLVKDYFPEPVTVSWNSGALTSGVHTFPAVLQSSGLYSLSSVVTVPSSSLGTQTYICNVNHKPSNTKVDKKVEPKSCDKTHTCPPCPAPELLGGPSVFLFPPKPKDTLMISRTPEVTCVVVDVSHEDPEVKFNWYVDGVEVHNAKTKPREEQYNSTYRVVSVLTVLHQDWLNGKEYKCKVSNKALPAPIEKTISKAKGQPREPQVYTLPPSRDELTKNQVSLTCLVKGFYPSDIAVEWESNGQPENNYKTTPPVLDSDGSFFLYSKLTVDKSRWQQGNVFSCSVMHEALHNHYTQKSLSLSPGK

SEQ ID NO: 243 - protein, 666 aa, artificial sequence
  G4_14 IgG1 antibody sequence
ASNFMLTQPHSVSESPGKTVTISCTRSRGSIAGNYVHWYQQRPGRAPTTVIYRDKERPSGVPDRISGSIDSSSNSASLTISGLKTEDEADYYCQSYDSSTHVVFGGGTKLTVLGQPAAAPSVTLFPPSSEELQANKATLVCLISDFYPGAVTVAWKADSSPVKAGVETTTPSKQSNNKYAASSYLSLTPEQWKSHRSYSCQVTHEGSTVEKTVAPTECSEVQLVQSGAEVKKPGESLRISCKGSGYSFTSYWISWVRQMPGKGLEWMGRIDPSDSYTNYSPSFPGHVTISADKSISTAYLQWSSLKASDTAMYYCAADTAHGMDVWGRGTLVTVSSASTKGPSVFPLAPSSKSTSGGTAALGCLVKDYFPEPVTVSWNSGALTSGVHTFPAVLQSSGLYSLSSVVTVPSSSLGTQTYICNVNHKPSNTKVDKKVEPKSCDKTHTCPPCPAPELLGGPSVFLFPPKPKDTLMISRTPEVTCVVVDVSHEDPEVKFNWYVDGVEVHNAKTKPREEQYNSTYRVVSVLTVLHQDWLNGKEYKCKVSNKALPAPIEKTISKAKGQPREPQVYTLPPSRDELTKNQVSLTCLVKGFYPSDIAVEWESNGQPENNYKTTPPVLDSDGSFFLYSKLTVDKSRWQQGNVFSCSVMHEALHNHYTQKSLSLSPGK

SEQ ID NO: 244 - protein, 668 aa, artificial sequence
  G4_15 IgG1 antibody sequence
ASQSALTQPASVSGSPGQSITISCTGTSSDVGGYNYVSWYQQHPGKAPKLMIYDVSNRPSGVSNRFSGSKSGNTASLTISGLQAEDEADYYCSSYGSGSVFGTGTKLTVLGQPAAAPSVTLFPPSSEELQANKATLVCLISDFYPGAVTVAWKADSSPVKAGVETTTPSKQSNNKYAASSYLSLTPEQWKSHRSYSCQVTHEGSTVEKTVAPTECSEVQLVQSEAEVKKPGASVKVSCKASGYTFTRHYMHWVRQAPGQGLEWMGLINPSGSSTVYAQKFQGRVTLTRDTSTSTDYMELSSLRSEDTAVYYCARDNSHLDQVWWFDPWGQGTLVTVSSASTKGPSVFPLAPSSKSTSGGTAALGCLVKDYFPEPVTVSWNSGALTSGVHTFPAVLQSSGLYSLSSVVTVPSSSLGTQTYICNVNHKPSNTKVDKKVEPKSCDKTHTCPPCPAPELLGGPSVFLFPPKPKDTLMISRTPEVTCVVVDVSHEDPEVKFNWYVDGVEVHNAKTKPREEQYNSTYRVVSVLTVLHQDWLNGKEYKCKVSNKALPAPIEKTISKAKGQPREPQVYTLPPSRDELTKNQVSLTCLVKGFYPSDIAVEWESNGQPENNYKTTPPVLDSDGSFFLYSKLTVDKSRWQQGNVFSCSVMHEALHNHYTQKSLSLSPGK

SEQ ID NO: 245 - protein, 667 aa, artificial sequence
  G4_16 IgG1 antibody sequence
ASQSVLTQPPSASGSPGQSVTFSCTGTSSDIGAFNSVSWYQQHPGKAPKLLIYEITKRPSGVPDRFSGSKSGNTASLTISVLQAEDEADYYCTSYAGSNTLIFGGGTKVTVLGQPAAAPSVTLFPPSSEELQANKATLVCLISDFYPGAVTVAWKADSSPVKAGVETTTPSKQSNNKYAASSYLSLTPEQWKSHRSYSCQVTHEGSTVEKTVAPTECSEVQLLESGAEVKKPGASVKVSCKASGYTFTSYGISWVRQAPGQGLEWMGWISAYNGNTNYAQKLQGRVTMTTDTSTSTAYMELRSLRSDDTAVYYCARDYGDFYGMDVWGQGTLVTVSSASTKGPSVFPLAPSSKSTSGGTAALGCLVKDYFPEPVTVSWNSGALTSGVHTFPAVLQSSGLYSLSSVVTVPSSSLGTQTYICNVNHKPSNTKVDKKVEPKSCDKTHTCPPCPAPELLGGPSVFLFPPKPKDTLMISRTPEVTCVVVDVSHEDPEVKFNWYVDGVEVHNAKTKPREEQYNSTYRVVSVLTVLHQDWLNGKEYKCKVSNKALPAPIEKTISKAKGQPREPQVYTLPPSRDELTKNQVSLTCLVKGFYPSDIAVEWESNGQPENNYKTTPPVLDSDGSFFLYSKLTVDKSRWQQGNVFSCSVMHEALHNHYTQKSLSLSPGK

SEQ ID NO: 246 - protein, 664 aa, artificial sequence
  G4_18 IgG1 antibody sequence
ASSYELTQPPSVTESPGQTARITCSGDALAKQYAYWYQQKPGQAPVLVIYRDSERPSEIPERFSGSSSGTTVTLTISGVQAEDEADYYCQSADSSGTYTVFGGGTKLTVLGQPAAAPSVTLFPPSSEELQANKATLVCLISDFYPGAVTVAWKADSSPVKAGVETTTPSKQSNNKYAASSYLSLTPEQWKSHRSYSCQVTHEGSTVEKTVAPTECSEVQLVESGAEVKKPGASVKVSCKASGYTFTGYYMHWVRQAPGQGLEWMGRINPNSGGTNYAQKFQGRVTMTRDASISTAYMELSRLRSDDTAVYYCARDLDLSSLDYWGRGTLVTVSSASTKGPSVFPLAPSSKSTSGGTAALGCLVKDYFPEPVTVSWNSGALTSGVHTFPAVLQSSGLYSLSSVVTVPSSSLGTQTYICNVNHKPSNTKVDKKVEPKSCDKTHTCPPCPAPELLGGPSVFLFPPKPKDTLMISRTPEVTCVVVDVSHEDPEVKFNWYVDGVEVHNAKTKPREEQYNSTYRVVSVLTVLHQDWLNGKEYKCKVSNKALPAPIEKTISKAKGQPREPQVYTLPPSRDELTKNQVSLTCLVKGFYPSDIAVEWESNGQPENNYKTTPPVLDSDGSFFLYSKLTVDKSRWQQGNVFSCSVMHEALHNHYTQKSLSLSPGK

SEQ ID NO: 247 - protein, 670 aa, artificial sequence
  G4_19 IgG1 antibody sequence
ASNFMLTQPHSVSESPGKTVTISCTRSSGSIASNYVQWYQQRPGSPPITLIYDDDQRPSGVPHRFSGSIDTSSNPASLTISGLKTEDEADYYCQSYDSSNHVVFGGGTKLTVLGQPAAAPSVTLFPPSSEELQANKATLVCLISDFYPGAVTVAWKADSSPVKAGVETTTPSKQSNNKYAASSYLSLTPEQWKSHRSYSCQVTHEGSTVEKTVAPTECSEVQLVQSGAEVKKPGASVKVSCKASGYTLTSYYMHWVRQAPGQGLEWMGIINPSGGSTSYAQKFQGRVTMTRDTSTSTVYMELSSLRSEDTAVYYCARERGYSYGDGMDVWGQGTTVTVSSASTKGPSVFPLAPSSKSTSGGTAALGCLVKDYFPEPVTVSWNSGALTSGVHTFPAVLQSSGLYSLSSVVTVPSSSLGTQTYICNVNHKPSNTKVDKKVEPKSCDKTHTCPPCPAPELLGGPSVFLFPPKPKDTLMISRTPEVTCVVVDVSHEDPEVKFNWYVDGVEVHNAKTKPREEQYNSTYRVVSVLTVLHQDWLNGKEYKCKVSNKALPAPIEKTISKAKGQPREPQVYTLPPSRDELTKNQVSLTCLVKGFYPSDIAVEWESNGQPENNYKTTPPVLDSDGSFFLYSKLTVDKSRWQQGNVFSCSVMHEALHNHYTQKSLSLSPGK

SEQ ID NO: 248 - protein, 663 aa, artificial sequence
  G4_20 IgG1 antibody sequence
ASSYELTHPPSVSVSPGQTASITCSGDKLGDKFVSWYHQKPGQSPVLVIYQDSKRPSGIPERFSGSNSGNTATLTISGTRAMDEADYYCQAWDSSTVVFGGGTKLTVLGQPAAAPSVTLFPPSSEELQANKATLVCLISDFYPGAVTVAWKADSSPVKAGVETTTPSKQSNNKYAASSYLSLTPEQWKSHRSYSCQVTHEGSTVEKTVAPTECSQVQLVESGAEVKKPGASVKVSCKASGGTFSSYAISWVRQAPGQGLEWMGGIIPIFGTANYAQKFQGRVTITVDKSTRTAYMELSSLRSKDTAVYYCARGNSRSDAFDIWGQGTMVTVSSASTKGPSVFPLAPSSKSTSGGTAALGCLVKDYFPEPVTVSWNSGALTSGVHTFPAVLQSSGLYSLSSVVTVPSSSLGTQTYICNVNHKPSNTKVDKKVEPKSCDKTHTCPPCPAPELLGGPSVFLFPPKPKDTLMISRTPEVTCVVVDVSHEDPEVKFNWYVDGVEVHNAKTKPREEQYNSTYRVVSVLTVLHQDWLNGKEYKCKVSNKALPAPIEKTISKAKGQPREPQVYTLPPSRDELTKNQVSLTCLVKGFYPSDIAVEWESNGQPENNYKTTPPVLDSDGSFFLYSKLTVDKSRWQQGNVFSCSVMHEALHNHYTQKSLSLSPGK

SEQ ID NO: 249 - protein, 666 aa, artificial sequence
  G4_22 IgG1 antibody sequence
ASDIQMTQSPSSLSASVGDRVTITCQASQDISNYLNWYQQKPGKAPKLLIYAASSLQSGVPSRFSVSGSGTDFTLTISNLQPEDFATYYCQQSYSIPWTFGQGTKVEIKRTAAAPSVFIFPPSDEQLKSGTASVVCLLNNFYPREAKVQWKVDNALQSGNSQESVTEQDSKDSTYSLSSTLTLSKADYEKHKLYACEVTHQGLSSPVTKSFNRGECQVQLVESGGGLVQPGGSLRLSCAASGFTFSTYAMSWVRQAPGKGLEWVSTVSGSGGTTYYADSVKGRFTISRDNSKNTLYLQMNSLRAEDTAVYYCAKDSTAVTDWFDPWGRGTLVTVSSASTKGPSVFPLAPSSKSTSGGTAALGCLVKDYFPEPVTVSWNSGALTSGVHTFPAVLQSSGLYSLSSVVTVPSSSLGTQTYICNVNHKPSNTKVDKKVEPKSCDKTHTCPPCPAPELLGGPSVFLFPPKPKDTLMISRTPEVTCVVVDVSHEDPEVKFNWYVDGVEVHNAKTKPREEQYNSTYRVVSVLTVLHQDWLNGKEYKCKVSNKALPAPIEKTISKAKGQPREPQVYTLPPSRDELTKNQVSLTCLVKGFYPSDIAVEWESNGQPENNYKTTPPVLDSDGSFFLYSKLTVDKSRWQQGNVFSCSVMHEALHNHYTQKSLSLSPGK

SEQ ID NO: 250 - protein, 666 aa, artificial sequence
  G4_23 IgG1 antibody sequence
ASDIQMTQSPSSLSASVGDRVTITCRASQGISNSLAWYQQKPGKAPKLLLYAASRLESGVPSRFSGSGSGTDYTLTISSLQPEDFATYYCQQYYSTPRTFGGGTKLEIKRTAAAPSVFIFPPSDEQLKSGTASVVCLLNNFYPREAKVQWKVDNALQSGNSQESVTEQDSKDSTYSLSSTLTLSKADYEKHKLYACEVTHQGLSSPVTKSFNRGECEVQLVESGGGVVQPGRSLRLSCAASGFTFSSYGMHWVRQAPGKGLEWVAVIWYDGSNKYYADSVKGRFTISRDNSKNTLYLQMNSLRAEDTAVYYCARGEVAALYYFDYWGQGTLVTVSSASTKGPSVFPLAPSSKSTSGGTAALGCLVKDYFPEPVTVSWNSGALTSGVHTFPAVLQSSGLYSLSSVVTVPSSSLGTQTYICNVNHKPSNTKVDKKVEPKSCDKTHTCPPCPAPELLGGPSVFLFPPKPKDTLMISRTPEVTCVVVDVSHEDPEVKFNWYVDGVEVHNAKTKPREEQYNSTYRVVSVLTVLHQDWLNGKEYKCKVSNKALPAPIEKTISKAKGQPREPQVYTLPPSRDELTKNQVSLTCLVKGFYPSDIAVEWESNGQPENNYKTTPPVLDSDGSFFLYSKLTVDKSRWQQGNVFSCSVMHEALHNHYTQKSLSLSPGK

SEQ ID NO: 251 - protein, 674 aa, artificial sequence
  G4_24 IgG1 antibody sequence
ASDIVMTQSPDSLAVSLGERATINCKSSQSVLYSSNNKNYLAWYQQKPGQPPKLLISWASTRESGVPDRFSGSGSGTDFTLTINSLQSEDVAIYYCQQYYSTPPTFGQGTKLEIKRTAAAPSVFIFPPSDEQLKSGTASVVCLLNNFYPREAKVQWKVDNALQSGNSQESVTEQDSKDSTYSLSSTLTLSKADYEKHKLYACEVTHQGLSSPVTKSFNRGECQVQLQQSGPGLVKPSQTLSLTCAISGASVSSNSVAWNWIRQSPSRGLEWLGRTYYRSRWYNDYALSVKSRIIINPDTSKNQFSLQLNSVTPEDTAVYYCARDWSSTRSFDYWGRGTLVTVSSASTKGPSVFPLAPSSKSTSGGTAALGCLVKDYFPEPVTVSWNSGALTSGVHTFPAVLQSSGLYSLSSVVTVPSSSLGTQTYICNVNHKPSNTKVDKKVEPKSCDKTHTCPPCPAPELLGGPSVFLFPPKPKDTLMISRTPEVTCVVVDVSHEDPEVKFNWYVDGVEVHNAKTKPREEQYNSTYRVVSVLTVLHQDWLNGKEYKCKVSNKALPAPIEKTISKAKGQPREPQVYTLPPSRDELTKNQVSLTCLVKGFYPSDIAVEWESNGQPENNYKTTPPVLDSDGSFFLYSKLTVDKSRWQQGNVFSCSVMHEALHNHYTQKSLSLSPGK

SEQ ID NO: 252 - protein, 669 aa, artificial sequence
  G4_25 IgG1 antibody sequence
ASQSALTQPRSVSGSPGQSVTISCTGTSSDVGGYNYVSWYQQHPGKAPKLMIYEVSNRPSGVSNRFSGSKSGNTASLTISGLQAEDEADYYCSSYGSGSVFGTGTKLTVLGQPAAAPSVTLFPPSSEELQANKATLVCLISDFYPGAVTVAWKADSSPVKAGVETTTPSKQSNNKYAASSYLSLTPEQWKSHRSYSCQVTHEGSTVEKTVAPTECSEVQLVESGAEVKKPGSSVKVSCKASGGTFSSYAISWVRQAPGQGLEWMGGIIPIFGTANYAQKFQGRVTITADKSTSTAYMELSSLRSEDTAVYYCARSLRDGYNYIGSLGYWGQGTLVTVSSASTKGPSVFPLAPSSKSTSGGTAALGCLVKDYFPEPVTVSWNSGALTSGVHTFPAVLQSSGLYSLSSVVTVPSSSLGTQTYICNVNHKPSNTKVDKKVEPKSCDKTHTCPPCPAPELLGGPSVFLFPPKPKDTLMISRTPEVTCVVVDVSHEDPEVKFNWYVDGVEVHNAKTKPREEQYNSTYRVVSVLTVLHQDWLNGKEYKCKVSNKALPAPIEKTISKAKGQPREPQVYTLPPSRDELTKNQVSLTCLVKGFYPSDIAVEWESNGQPENNYKTTPPVLDSDGSFFLYSKLTVDKSRWQQGNVFSCSVMHEALHNHYTQKSLSLSPGK

SEQ ID NO: 253 - protein, 666 aa, artificial sequence
  G4_26 IgG1 antibody sequence
ASQSGLTQPASVSGSPGQSITISCTGTSSDVGSYNLVSWYQQHPGKAPKLMIYEVSKRPSGVSNRFSGSKSGNTASLTISGLQAEDEADYYCSSFGSGSIFGTGTKLTVLGQPAAAPSVTLFPPSSEELQANKATLVCLISDFYPGAVTVAWKADSSPVKAGVETTTPSKQSNNKYAASSYLSLTPEQWKSHRSYSCQVTHEGSTVEKTVAPTECSQVQLVQSGAEVKKPGSSVKVSCKASGGTFSSYAISWVRQAPGQGLEWMGGIIPIFGTANYAQKFQGRVTITADESTSTAYMELSSLRSEDTAVYYCASSRGSGWFPLGYWGQGTLVTVSSASTKGPSVFPLAPSSKSTSGGTAALGCLVKDYFPEPVTVSWNSGALTSGVHTFPAVLQSSGLYSLSSVVTVPSSSLGTQTYICNVNHKPSNTKVDKKVEPKSCDKTHTCPPCPAPELLGGPSVFLFPPKPKDTLMISRTPEVTCVVVDVSHEDPEVKFNWYVDGVEVHNAKTKPREEQYNSTYRVVSVLTVLHQDWLNGKEYKCKVSNKALPAPIEKTISKAKGQPREPQVYTLPPSRDELTKNQVSLTCLVKGFYPSDIAVEWESNGQPENNYKTTPPVLDSDGSFFLYSKLTVDKSRWQQGNVFSCSVMHEALHNHYTQKSLSLSPGK

SEQ ID NO: 254 - protein, 668 aa, artificial sequence
  G4_27 IgG1 antibody sequence
ASSYELTQDPAVSVALGQTVSITCQGDSLRNFYANWYQQKPGQAPVLVIYGKNNRPSGIPDRFSGSSSGNTASLTITGAQAEDEADYYCNSRDSSGNHLVFGGGTQLTVLGQPAAAPSVTLFPPSSEELQANKATLVCLISDFYPGAVTVAWKADSSPVKAGVETTTPSKQSNNKYAASSYLSLTPEQWKSHRSYSCQVTHEGSTVEKTVAPTECSQVQLVQSGAEVKKPGESLKISCKSSGYSFTSYWIGWVRQMPGKGLEWMGIIYPGDSDTRYSPSFQGQVTFSADESISTAYLQWSSLKASDTAMYYCARHGAYGDYPDTFDIWGQGTLVTVSSASTKGPSVFPLAPSSKSTSGGTAALGCLVKDYFPEPVTVSWNSGALTSGVHTFPAVLQSSGLYSLSSVVTVPSSSLGTQTYICNVNHKPSNTKVDKKVEPKSCDKTHTCPPCPAPELLGGPSVFLFPPKPKDTLMISRTPEVTCVVVDVSHEDPEVKFNWYVDGVEVHNAKTKPREEQYNSTYRVVSVLTVLHQDWLNGKEYKCKVSNKALPAPIEKTISKAKGQPREPQVYTLPPSRDELTKNQVSLTCLVKGFYPSDIAVEWESNGQPENNYKTTPPVLDSDGSFFLYSKLTVDKSRWQQGNVFSCSVMHEALHNHYTQKSLSLSPGK

SEQ ID NO: 255 - protein, 669 aa, artificial sequence
  G4_28 IgG1 antibody sequence
ASSYELTQDPAVSVALGQTVTITCQGDSLRNYYASWYRQKPGQTPVLVVYGKNNRPSGIPDRFSVSASGNTASLTITGAQAEDEGDYYCNSRDSSGVVFGGGTKVTVLGQPAAAPSVTLFPPSSEELQANKATLVCLISDFYPGAVTVAWKADSSPVKAGVETTTPSKQSNNKYAASSYLSLTPEQWKSHRSYSCQVTHEGSTVEKTVAPTECSQVQLVESGGGLVQPGGSLRLSCAASGFTFDDYAMHWVRQAPGKGLEWVSGISAGGGSTNYAGSVKGRFTVSRDTSKNTLYLQMNSLRAEDTAVYYCVKSYVDTAMRYYYYYMDVWGQGTMVTVSSASTKGPSVFPLAPSSKSTSGGTAALGCLVKDYFPEPVTVSWNSGALTSGVHTFPAVLQSSGLYSLSSVVTVPSSSLGTQTYICNVNHKPSNTKVDKKVEPKSCDKTHTCPPCPAPELLGGPSVFLFPPKPKDTLMISRTPEVTCVVVDVSHEDPEVKFNWYVDGVEVHNAKTKPREEQYNSTYRVVSVLTVLHQDWLNGKEYKCKVSNKALPAPIEKTISKAKGQPREPQVYTLPPSRDELTKNQVSLTCLVKGFYPSDIAVEWESNGQPENNYKTTPPVLDSDGSFFLYSKLTVDKSRWQQGNVFSCSVMHEALHNHYTQKSLSLSPGK

SEQ ID NO: 256 - protein, 270 aa, artificial sequence
  TRGV4(4MNH) TRAC antigen sequence
SSNLEGRTKSVIRQTGSSAEITCDLAEGSTGYIHWYLHQEGKAPQRLLYYDSYTSSVVLESGISPGKYDTYGSTRKNLRMILRNLIENDSGVYYCATWDEKYYKKLFGSGTTLVVTEDLKNVFPPEVAVFEPSEAEISHTQKATLVCLATGFYPDHVELSWWVNGKEVHSGVSTDPQPLKEQPALNDSRYALSSRLRVSATFWQNPRNHFRCQVQFYGLSENDEWTQDRAKPVTQIVSAEAWGRADCTTAPSAQLEKELQALEKENAQLE

SEQ ID NO: 257 - protein, 282 aa, artificial sequence
  V gamma 4 (4MNH) GV4TRBC leucine zipper heterodimer antigen sequence
SSNLEGRTKSVIRQTGSSAEITCDLAEGSTGYIHWYLHQEGKAPQRLLYYDSYTSSVVLESGISPGKYDTYGSTRKNLRMILRNLIENDSGVYYCATWDEKYYKKLFGSGTTLVVTEDLKNVFPPEVAVFEPSEAEISHTQKATLVCLATGFYPDHVELSWWVNGKEVHSGVSTDPQPLKEQPALNDSRYALSSRLRVSATFWQNPRNHFRCQVQFYGLSENDEWTQDRAKPVTQIVSAEAWGRADCTTAPSAQLEKELQALEKENAQLEWELQALEKELAQ

SEQ ID NO: 258 - protein, 348 aa, artificial sequence
  V gamma 4 TRGV4(4MNH) Fc heterodimer antigen sequence
SSNLEGRTKSVIRQTGSSAEITCDLAEGSTGYIHWYLHQEGKAPQRLLYYDSYTSSVVLESGISPGKYDTYGSTRKNLRMILRNLIENDSGVYYCATWDEKYYKKLFGSGTTLVVTEDAAADKTHTCPPCPAPELLGGPSVFLFPPKPKDTLMISRTPEVTCVVVDVSHEDPEVKFNWYVDGVEVHNAKTKPREEQYNSTYRVVSVLTVLHQDWLNGKEYKCKVSNKALPAPIEKTISKAKGQPREPQVYTLPPSRDELTKNQVSLTCLVKGFYPSDIAVEWESNGQPENNYKTTPPVLDSDGSFFLYSKLTVDKSRWQQGNVFSCSVSHEALHSHHTQKSLSLSPGK

SEQ ID NO: 259 - protein, 282 aa, artificial sequence
  V gamma 2 (4MNH) GV2TRBC leucine zipper heterodimer antigen sequence
SSNLEGRTKSVIRQTGSSAEITCDLAEGSNGYIHWYLHQEGKAPQRLQYYDSYNSKVVLESGVSPGKYYTYASTRNNLRLILRNLIENDSGVYYCATWDEKYYKKLFGSGTTLVVTEDLKNVFPPEVAVFEPSEAEISHTQKATLVCLATGFYPDHVELSWWVNGKEVHSGVSTDPQPLKEQPALNDSRYALSSRLRVSATFWQNPRNHFRCQVQFYGLSENDEWTQDRAKPVTQIVSAEAWGRADCTTAPSAQLEKELQALEKENAQLEWELQALEKELAQ

SEQ ID NO: 260 - protein, 348 aa, artificial sequence
  V gamma 2 TRGV2(4MNH) Fc heterodimer antigen sequence
SSNLEGRTKSVIRQTGSSAEITCDLAEGSNGYIHWYLHQEGKAPQRLQYYDSYNSKVVLESGVSPGKYYTYASTRNNLRLILRNLIENDSGVYYCATWDEKYYKKLFGSGTTLVVTEDAAADKTHTCPPCPAPELLGGPSVFLFPPKPKDTLMISRTPEVTCVVVDVSHEDPEVKFNWYVDGVEVHNAKTKPREEQYNSTYRVVSVLTVLHQDWLNGKEYKCKVSNKALPAPIEKTISKAKGQPREPQVYTLPPSRDELTKNQVSLTCLVKGFYPSDIAVEWESNGQPENNYKTTPPVLDSDGSFFLYSKLTVDKSRWQQGNVFSCSVSHEALHSHHTQKSLSLSPGK

SEQ ID NO: 261 - protein, 107 aa, artificial sequence
  TRGV4 full light variable sequence G4_1 no N-terminal AS
DIQMTQSPSSLSASVGDRVTITCQASQDISNYLNWYQQKPGKAPKLLIYDASNLETGVPSRFSGSGSGTDFTLTISSLQPEDFATYYCQQSYSTPVTFGPGTKVEIK

SEQ ID NO: 262 - protein, 107 aa, artificial sequence
  TRGV4 full light variable sequence G4_2 no N-terminal AS
DIQMTQSPSSLSASVGDRVTITCQASQDISNYLNWYQQKPGKAPKLLIYAASSLQSGVPSRFSGSGSGTDFTLTISGLQPEDFATYYCLEDYNYLWTFGQGTKLEIK

SEQ ID NO: 263 - protein, 107 aa, artificial sequence
  TRGV4 full light variable sequence G4_3 no N-terminal AS
DIQMTQSPSSLSASVGDRVTITCQASQDISNYLNWYQQKPGKAPKLLIYDASNLETGVPSRFSGSGSGTDFTLTISSLQPEDFATYFCQQSYSTPQTFGQGTKVDIK

SEQ ID NO: 264 - protein, 113 aa, artificial sequence
  TRGV4 full light variable sequence G4_4 no N-terminal AS
DIVMTQSPDSLAVSLGERATINCKSSQSVLSSSNNNNYLAWYQQRPGQPPKLLFYWASTRESGVPDRFSGSGSGTSFTLTITSLQAEDVAVYYCQQYYSTPLTFGGGTKLEIK

SEQ ID NO: 265 - protein, 107 aa, artificial sequence
  TRGV4 full light variable sequence G4_5 no N-terminal AS
DIQMTQSPSSLSASVGDRVTITCRASQSISSYLNWYQQKPGKAPKLLIYAASSLQSGVPSRFSGSGSGTDFTLTISSLQPEDFATYYCQQSYSTPYTFGQGTKVEIK

SEQ ID NO: 266 - protein, 107 aa, artificial sequence
  TRGV4 full light variable sequence G4_6 no N-terminal AS
DIQMTQSPSSLSASVGDRVTITCRASQSISTYLNWYQQKPGKAPKLLIYAASSLQSGVPSRFSGSGSGTDFTLTISSPQPEDFATYYCQQSYSTPYTFGQGTKVEIK

SEQ ID NO: 267 - protein, 112 aa, artificial sequence
  TRGV4 full light variable sequence G4_7 no N-terminal AS
DIVMTQSPLSLPVTPGEPASISCRSSQSLLHSNRFNYLDWYLQKPGQSPQLLIYLGSNRASGVPDRFSGSGSGTDFTLKISRVEAEDVGVYYCMQGLQTPYTFGQGTKVDIK

SEQ ID NO: 268 - protein, 112 aa, artificial sequence
  TRGV4 full light variable sequence G4_10 no N-terminal AS
DIVMTQPPLSLPVTLGHPASISCKSSQSLEYSDGNTYLNWFQQRPGQSPRRLIYKVSNRDSGAPDRFSGSGSGTDFTLEISRVEAEDVGVYYCMQGTLWPPTFGQGTKVDIK

SEQ ID NO: 269 - protein, 108 aa, artificial sequence
  TRGV4 full light variable sequence G4_12 no N-terminal AS
QSVLTQPASVSGSPGQSITISCTGTSSDVGGYNFVSWYQQHPGKAPKLMIYEVTNRPSGVPDRFSGSKSGNTASLTISGLQAEDEADYYCSSHASPRVFGTGTKVTVL

SEQ ID NO: 270 - protein, 111 aa, artificial sequence
  TRGV4 full light variable sequence G4_13 no N-terminal AS
NFMLTQPHSVSESPGKTVTISCTRSSGSIASNYVQWYQQRPGSSPSTVIYEDNQRPSGVPDRFSGSIDSSSNSASLTISGLRTEDEADYYCQSYDSSIYVVFGGGTKLTVL

SEQ ID NO: 271 - protein, 111 aa, artificial sequence
  TRGV4 full light variable sequence G4_14 no N-terminal AS
NFMLTQPHSVSESPGKTVTISCTRSRGSIAGNYVHWYQQRPGRAPTTVIYRDKERPSGVPDRISGSIDSSSNSASLTISGLKTEDEADYYCQSYDSSTHVVFGGGTKLTVL

SEQ ID NO: 272 - protein, 108 aa, artificial sequence
  TRGV4 full light variable sequence G4_15 no N-terminal AS
QSALTQPASVSGSPGQSITISCTGTSSDVGGYNYVSWYQQHPGKAPKLMIYDVSNRPSGVSNRFSGSKSGNTASLTISGLQAEDEADYYCSSYGSGSVFGTGTKLTVL

SEQ ID NO: 273 - protein, 110 aa, artificial sequence
  TRGV4 full light variable sequence G4_16 no N-terminal AS
QSVLTQPPSASGSPGQSVTFSCTGTSSDIGAFNSVSWYQQHPGKAPKLLIYEITKRPSGVPDRFSGSKSGNTASLTISVLQAEDEADYYCTSYAGSNTLIFGGGTKVTVL

SEQ ID NO: 274 - protein, 108 aa, artificial sequence
  TRGV4 full light variable sequence G4_18 no N-terminal AS
SYELTQPPSVTESPGQTARITCSGDALAKQYAYWYQQKPGQAPVLVIYRDSERPSEIPERFSGSSSGTTVTLTISGVQAEDEADYYCQSADSSGTYTVFGGGTKLTVL

SEQ ID NO: 275 - protein, 111 aa, artificial sequence
  TRGV4 full light variable sequence G4_19 no N-terminal AS
NFMLTQPHSVSESPGKTVTISCTRSSGSIASNYVQWYQQRPGSPPITLIYDDDQRPSGVPHRFSGSIDTSSNPASLTISGLKTEDEADYYCQSYDSSNHVVFGGGTKLTVL

SEQ ID NO: 276 - protein, 106 aa, artificial sequence
  TRGV4 full light variable sequence G4_20 no N-terminal AS
SYELTHPPSVSVSPGQTASITCSGDKLGDKFVSWYHQKPGQSPVLVIYQDSKRPSGIPERFSGSNSGNTATLTISGTRAMDEADYYCQAWDSSTVVFGGGTKLTVL

SEQ ID NO: 277 - protein, 107 aa, artificial sequence
  TRGV4 full light variable sequence G4_22 no N-terminal AS
DIQMTQSPSSLSASVGDRVTITCQASQDISNYLNWYQQKPGKAPKLLIYAASSLQSGVPSRFSVSGSGTDFTLTISNLQPEDFATYYCQQSYSIPWTFGQGTKVEIK

SEQ ID NO: 278 - protein, 107 aa, artificial sequence
  TRGV4 full light variable sequence G4_23 no N-terminal AS
DIQMTQSPSSLSASVGDRVTITCRASQGISNSLAWYQQKPGKAPKLLLYAASRLESGVPSRFSGSGSGTDYTLTISSLQPEDFATYYCQQYYSTPRTFGGGTKLEIK

SEQ ID NO: 279 - protein, 113 aa, artificial sequence
  TRGV4 full light variable sequence G4_24 no N-terminal AS
DIVMTQSPDSLAVSLGERATINCKSSQSVLYSSNNKNYLAWYQQKPGQPPKLLISWASTRESGVPDRFSGSGSGTDFTLTINSLQSEDVAIYYCQQYYSTPPTFGQGTKLEIK

SEQ ID NO: 280 - protein, 108 aa, artificial sequence
  TRGV4 full light variable sequence G4_25 no N-terminal AS
QSALTQPRSVSGSPGQSVTISCTGTSSDVGGYNYVSWYQQHPGKAPKLMIYEVSNRPSGVSNRFSGSKSGNTASLTISGLQAEDEADYYCSSYGSGSVFGTGTKLTVL

SEQ ID NO: 281 - protein, 108 aa, artificial sequence
  TRGV4 full light variable sequence G4_26 no N-terminal AS
QSGLTQPASVSGSPGQSITISCTGTSSDVGSYNLVSWYQQHPGKAPKLMIYEVSKRPSGVSNRFSGSKSGNTASLTISGLQAEDEADYYCSSFGSGSIFGTGTKLTVL

SEQ ID NO: 282 - protein, 108 aa, artificial sequence
  TRGV4 full light variable sequence G4_27 no N-terminal AS
SYELTQDPAVSVALGQTVSITCQGDSLRNFYANWYQQKPGQAPVLVIYGKNNRPSGIPDRFSGSSSGNTASLTITGAQAEDEADYYCNSRDSSGNHLVFGGGTQLTVL

SEQ ID NO: 283 - protein, 106 aa, artificial sequence
  TRGV4 full light variable sequence G4_28 no N-terminal AS
SYELTQDPAVSVALGQTVTITCQGDSLRNYYASWYRQKPGQTPVLVVYGKNNRPSGIPDRFSVSASGNTASLTITGAQAEDEGDYYCNSRDSSGVVFGGGTKVTVL

SEQ ID NO: 284 - protein, 446 aa, artificial sequence
  G4_1 IgG1 antibody heavy chain sequence
EVQLLESGGGVVQPGRPLRLSCAASGFTFSSYSMNWVRQAPGKGLEWVSSISSSSSYIYYADSVKGRFTISRDNSKNTLYLQMNSLRAEDTAVYYCAKGHWYFDLWGRGTLVTVSSASTKGPSVFPLAPSSKSTSGGTAALGCLVKDYFPEPVTVSWNSGALTSGVHTFPAVLQSSGLYSLSSVVTVPSSSLGTQTYICNVNHKPSNTKVDKKVEPKSCDKTHTCPPCPAPELLGGPSVFLFPPKPKDTLMISRTPEVTCVVVDVSHEDPEVKFNWYVDGVEVHNAKTKPREEQYNSTYRVVSVLTVLHQDWLNGKEYKCKVSNKALPAPIEKTISKAKGQPREPQVYTLPPSRDELTKNQVSLTCLVKGFYPSDIAVEWESNGQPENNYKTTPPVLDSDGSFFLYSKLTVDKSRWQQGNVFSCSVMHEALHNHYTQKSLSLSPGK

SEQ ID NO: 285 - protein, 450 aa, artificial sequence
  G4_2 IgG1 antibody heavy chain sequence
QMQLVQSGAEVKKPGATVKISCKVSGYPFTDYYIHWVQQAPGKGLEWMGLVDPEDGQSRSAERFQGRVTITADTSTDTAYMELSSLRSEDTAVYYCATFPVAGFYGMDVWGQGTLVTVSSASTKGPSVFPLAPSSKSTSGGTAALGCLVKDYFPEPVTVSWNSGALTSGVHTFPAVLQSSGLYSLSSVVTVPSSSLGTQTYICNVNHKPSNTKVDKKVEPKSCDKTHTCPPCPAPELLGGPSVFLFPPKPKDTLMISRTPEVTCVVVDVSHEDPEVKFNWYVDGVEVHNAKTKPREEQYNSTYRVVSVLTVLHQDWLNGKEYKCKVSNKALPAPIEKTISKAKGQPREPQVYTLPPSRDELTKNQVSLTCLVKGFYPSDIAVEWESNGQPENNYKTTPPVLDSDGSFFLYSKLTVDKSRWQQGNVFSCSVMHEALHNHYTQKSLSLSPGK

SEQ ID NO: 286 - protein, 446 aa, artificial sequence
  G4_3 IgG1 antibody heavy chain sequence
EVQLVESGGGLVQPGGSLRLSCAASGFTFSSYSMNWVRQAPGKGLEWVSSISSSSSYIYYADSVKGRFTISRDNSKNTLYLQMNSLRAEDTAVYYCARGGWLYDYWGQGTLVTVSSASTKGPSVFPLAPSSKSTSGGTAALGCLVKDYFPEPVTVSWNSGALTSGVHTFPAVLQSSGLYSLSSVVTVPSSSLGTQTYICNVNHKPSNTKVDKKVEPKSCDKTHTCPPCPAPELLGGPSVFLFPPKPKDTLMISRTPEVTCVVVDVSHEDPEVKFNWYVDGVEVHNAKTKPREEQYNSTYRVVSVLTVLHQDWLNGKEYKCKVSNKALPAPIEKTISKAKGQPREPQVYTLPPSRDELTKNQVSLTCLVKGFYPSDIAVEWESNGQPENNYKTTPPVLDSDGSFFLYSKLTVDKSRWQQGNVFSCSVMHEALHNHYTQKSLSLSPGK

SEQ ID NO: 287 - protein, 449 aa, artificial sequence
  G4_4 IgG1 antibody heavy chain sequence
QVQLVESGGGLVQPGGSLRLSCAASGFTFSSYAMSWVRQAPGKGLEWVSAISGSGGSTYYADSVKGRFTISRDNSKNTLYLQMSSLRVEDTAVYYCAKSSVGWWSFDYWGQGTMVTVSSASTKGPSVFPLAPSSKSTSGGTAALGCLVKDYFPEPVTVSWNSGALTSGVHTFPAVLQSSGLYSLSSVVTVPSSSLGTQTYICNVNHKPSNTKVDKKVEPKSCDKTHTCPPCPAPELLGGPSVFLFPPKPKDTLMISRTPEVTCVVVDVSHEDPEVKFNWYVDGVEVHNAKTKPREEQYNSTYRVVSVLTVLHQDWLNGKEYKCKVSNKALPAPIEKTISKAKGQPREPQVYTLPPSRDELTKNQVSLTCLVKGFYPSDIAVEWESNGQPENNYKTTPPVLDSDGSFFLYSKLTVDKSRWQQGNVFSCSVMHEALHNHYTQKSLSLSPGK

SEQ ID NO: 288 - protein, 450 aa, artificial sequence
  G4_5 IgG1 antibody heavy chain sequence
EVQLVQSGAEVKKPGSSVKVSCKASGYTFTSYGISWVRQAPGQGLEWMGWIGAYNGNTNYAQKLQGRVTMSTDTSTSTAYMELRSPRSDDTAVYYCARGGTGGDHVFAYWGQGTTVTVSSASTKGPSVFPLAPSSKSTSGGTAALGCLVKDYFPEPVTVSWNSGALTSGVHTFPAVLQSSGLYSLSSVVTVPSSSLGTQTYICNVNHKPSNTKVDKKVEPKSCDKTHTCPPCPAPELLGGPSVFLFPPKPKDTLMISRTPEVTCVVVDVSHEDPEVKFNWYVDGVEVHNAKTKPREEQYNSTYRVVSVLTVLHQDWLNGKEYKCKVSNKALPAPIEKTISKAKGQPREPQVYTLPPSRDELTKNQVSLTCLVKGFYPSDIAVEWESNGQPENNYKTTPPVLDSDGSFFLYSKLTVDKSRWQQGNVFSCSVMHEALHNHYTQKSLSLSPGK

SEQ ID NO: 289 - protein, 450 aa, artificial sequence
  G4_6 IgG1 antibody heavy chain sequence
EVQLVESGGGLVQPGGPLRLSCAASGFTFSSYAMNWVRQAPGKGLEWVSAISGSGGSTYYADSVKGRFTISRDNSKNTLYLQMNSLRAEDTAVYYCAKADYGVVYYFDYWGQGTMVTVSSASTKGPSVFPLAPSSKSTSGGTAALGCLVKDYFPEPVTVSWNSGALTSGVHTFPAVLQSSGLYSLSSVVTVPSSSLGTQTYICNVNHKPSNTKVDKKVEPKSCDKTHTCPPCPAPELLGGPSVFLFPPKPKDTLMISRTPEVTCVVVDVSHEDPEVKFNWYVDGVEVHNAKTKPREEQYNSTYRVVSVLTVLHQDWLNGKEYKCKVSNKALPAPIEKTISKAKGQPREPQVYTLPPSRDELTKNQVSLTCLVKGFYPSDIAVEWESNGQPENNYKTTPPVLDSDGSFFLYSKLTVDKSRWQQGNVFSCSVMHEALHNHYTQKSLSLSPGK

SEQ ID NO: 290 - protein, 449 aa, artificial sequence
  G4_7 IgG1 antibody heavy chain sequence
EVQLVESGGGWVQSGGSLRPSCAASGFTFSHYWMSWVRQAPGKGLEWVANIKQDGSIIYYADSVKGRFTISRDNAKNSVYLQMNSLRAEDTAVYYCARIGYSSSSFDYWGRGTLVTVSSASTKGPSVFPLAPSSKSTSGGTAALGCLVKDYFPEPVTVSWNSGALTSGVHTFPAVLQSSGLYSLSSVVTVPSSSLGTQTYICNVNHKPSNTKVDKKVEPKSCDKTHTCPPCPAPELLGGPSVFLFPPKPKDTLMISRTPEVTCVVVDVSHEDPEVKFNWYVDGVEVHNAKTKPREEQYNSTYRVVSVLTVLHQDWLNGKEYKCKVSNKALPAPIEKTISKAKGQPREPQVYTLPPSRDELTKNQVSLTCLVKGFYPSDIAVEWESNGQPENNYKTTPPVLDSDGSFFLYSKLTVDKSRWQQGNVFSCSVMHEALHNHYTQKSLSLSPGK

SEQ ID NO: 291 - protein, 452 aa, artificial sequence
  G4_10 IgG1 antibody heavy chain sequence
QVQLVESGGGVVQPGRPLRLSCAASGFTFSSYAMHWVRQAPGKGLEWVSAISGSGGSTYYADSVKGRFTISRDNSKNTLYLQMNSLRAEDTAVYYCAKDGAVDFWRNGMDVWGRGTLVTVSSASTKGPSVFPLAPSSKSTSGGTAALGCLVKDYFPEPVTVSWNSGALTSGVHTFPAVLQSSGLYSLSSVVTVPSSSLGTQTYICNVNHKPSNTKVDKKVEPKSCDKTHTCPPCPAPELLGGPSVFLFPPKPKDTLMISRTPEVTCVVVDVSHEDPEVKFNWYVDGVEVHNAKTKPREEQYNSTYRVVSVLTVLHQDWLNGKEYKCKVSNKALPAPIEKTISKAKGQPREPQVYTLPPSRDELTKNQVSLTCLVKGFYPSDIAVEWESNGQPENNYKTTPPVLDSDGSFFLYSKLTVDKSRWQQGNVFSCSVMHEALHNHYTQKSLSLSPGK

SEQ ID NO: 292 - protein, 447 aa, artificial sequence
  G4_12 IgG1 antibody heavy chain sequence
EVQLLESGGGLVQPGGSLRLSCAASGFTVSSNYMSWVRQAPGKGLEWVSVIYSGGSTYYADSVKGRFTISRHNSKNTLYLQMNSLRAEDTAVYYCARVANGDFLDYWGRGTLVTVSSASTKGPSVFPLAPSSKSTSGGTAALGCLVKDYFPEPVTVSWNSGALTSGVHTFPAVLQSSGLYSLSSVVTVPSSSLGTQTYICNVNHKPSNTKVDKKVEPKSCDKTHTCPPCPAPELLGGPSVFLFPPKPKDTLMISRTPEVTCVVVDVSHEDPEVKFNWYVDGVEVHNAKTKPREEQYNSTYRVVSVLTVLHQDWLNGKEYKCKVSNKALPAPIEKTISKAKGQPREPQVYTLPPSRDELTKNQVSLTCLVKGFYPSDIAVEWESNGQPENNYKTTPPVLDSDGSFFLYSKLTVDKSRWQQGNVFSCSVMHEALHNHYTQKSLSLSPGK

SEQ ID NO: 293 - protein, 447 aa, artificial sequence
  G4_13 IgG1 antibody heavy chain sequence
QVQLVESGAEVKKPGGSLRLSCAASGFTFSSYSMNWVRQAPGKGLEWVSSISGTSSYIYYADSVKGRFTISRDNAKNSLYLQMSSLRAEDTAVYYCARGGLGMVDPWGQGTLVTVSSASTKGPSVFPLAPSSKSTSGGTAALGCLVKDYFPEPVTVSWNSGALTSGVHTFPAVLQSSGLYSLSSVVTVPSSSLGTQTYICNVNHKPSNTKVDKKVEPKSCDKTHTCPPCPAPELLGGPSVFLFPPKPKDTLMISRTPEVTCVVVDVSHEDPEVKFNWYVDGVEVHNAKTKPREEQYNSTYRVVSVLTVLHQDWLNGKEYKCKVSNKALPAPIEKTISKAKGQPREPQVYTLPPSRDELTKNQVSLTCLVKGFYPSDIAVEWESNGQPENNYKTTPPVLDSDGSFFLYSKLTVDKSRWQQGNVFSCSVMHEALHNHYTQKSLSLSPGK

SEQ ID NO: 294 - protein, 447 aa, artificial sequence
  G4_14 IgG1 antibody heavy chain sequence
EVQLVQSGAEVKKPGESLRISCKGSGYSFTSYWISWVRQMPGKGLEWMGRIDPSDSYTNYSPSFPGHVTISADKSISTAYLQWSSLKASDTAMYYCAADTAHGMDVWGRGTLVTVSSASTKGPSVFPLAPSSKSTSGGTAALGCLVKDYFPEPVTVSWNSGALTSGVHTFPAVLQSSGLYSLSSVVTVPSSSLGTQTYICNVNHKPSNTKVDKKVEPKSCDKTHTCPPCPAPELLGGPSVFLFPPKPKDTLMISRTPEVTCVVVDVSHEDPEVKFNWYVDGVEVHNAKTKPREEQYNSTYRVVSVLTVLHQDWLNGKEYKCKVSNKALPAPIEKTISKAKGQPREPQVYTLPPSRDELTKNQVSLTCLVKGFYPSDIAVEWESNGQPENNYKTTPPVLDSDGSFFLYSKLTVDKSRWQQGNVFSCSVMHEALHNHYTQKSLSLSPGK

SEQ ID NO: 295 - protein, 452 aa, artificial sequence
  G4_15 IgG1 antibody heavy chain sequence
EVQLVQSEAEVKKPGASVKVSCKASGYTFTRHYMHWVRQAPGQGLEWMGLINPSGSSTVYAQKFQGRVTLTRDTSTSTDYMELSSLRSEDTAVYYCARDNSHLDQVWWFDPWGQGTLVTVSSASTKGPSVFPLAPSSKSTSGGTAALGCLVKDYFPEPVTVSWNSGALTSGVHTFPAVLQSSGLYSLSSVVTVPSSSLGTQTYICNVNHKPSNTKVDKKVEPKSCDKTHTCPPCPAPELLGGPSVFLFPPKPKDTLMISRTPEVTCVVVDVSHEDPEVKFNWYVDGVEVHNAKTKPREEQYNSTYRVVSVLTVLHQDWLNGKEYKCKVSNKALPAPIEKTISKAKGQPREPQVYTLPPSRDELTKNQVSLTCLVKGFYPSDIAVEWESNGQPENNYKTTPPVLDSDGSFFLYSKLTVDKSRWQQGNVFSCSVMHEALHNHYTQKSLSLSPGK

SEQ ID NO: 296 - protein, 449 aa, artificial sequence
  G4_16 IgG1 antibody heavy chain sequence
EVQLLESGAEVKKPGASVKVSCKASGYTFTSYGISWVRQAPGQGLEWMGWISAYNGNTNYAQKLQGRVTMTTDTSTSTAYMELRSLRSDDTAVYYCARDYGDFYGMDVWGQGTLVTVSSASTKGPSVFPLAPSSKSTSGGTAALGCLVKDYFPEPVTVSWNSGALTSGVHTFPAVLQSSGLYSLSSVVTVPSSSLGTQTYICNVNHKPSNTKVDKKVEPKSCDKTHTCPPCPAPELLGGPSVFLFPPKPKDTLMISRTPEVTCVVVDVSHEDPEVKFNWYVDGVEVHNAKTKPREEQYNSTYRVVSVLTVLHQDWLNGKEYKCKVSNKALPAPIEKTISKAKGQPREPQVYTLPPSRDELTKNQVSLTCLVKGFYPSDIAVEWESNGQPENNYKTTPPVLDSDGSFFLYSKLTVDKSRWQQGNVFSCSVMHEALHNHYTQKSLSLSPGK

SEQ ID NO: 297 - protein, 448 aa, artificial sequence
  G4_18 IgG1 antibody heavy chain sequence
EVQLVESGAEVKKPGASVKVSCKASGYTFTGYYMHWVRQAPGQGLEWMGRINPNSGGTNYAQKFQGRVTMTRDASISTAYMELSRLRSDDTAVYYCARDLDLSSLDYWGRGTLVTVSSASTKGPSVFPLAPSSKSTSGGTAALGCLVKDYFPEPVTVSWNSGALTSGVHTFPAVLQSSGLYSLSSVVTVPSSSLGTQTYICNVNHKPSNTKVDKKVEPKSCDKTHTCPPCPAPELLGGPSVFLFPPKPKDTLMISRTPEVTCVVVDVSHEDPEVKFNWYVDGVEVHNAKTKPREEQYNSTYRVVSVLTVLHQDWLNGKEYKCKVSNKALPAPIEKTISKAKGQPREPQVYTLPPSRDELTKNQVSLTCLVKGFYPSDIAVEWESNGQPENNYKTTPPVLDSDGSFFLYSKLTVDKSRWQQGNVFSCSVMHEALHNHYTQKSLSLSPGK

SEQ ID NO: 298 - protein, 451 aa, artificial sequence
  G4_19 IgG1 antibody heavy chain sequence
EVQLVQSGAEVKKPGASVKVSCKASGYTLTSYYMHWVRQAPGQGLEWMGIINPSGGSTSYAQKFQGRVTMTRDTSTSTVYMELSSLRSEDTAVYYCARERGYSYGDGMDVWGQGTTVTVSSASTKGPSVFPLAPSSKSTSGGTAALGCLVKDYFPEPVTVSWNSGALTSGVHTFPAVLQSSGLYSLSSVVTVPSSSLGTQTYICNVNHKPSNTKVDKKVEPKSCDKTHTCPPCPAPELLGGPSVFLFPPKPKDTLMISRTPEVTCVVVDVSHEDPEVKFNWYVDGVEVHNAKTKPREEQYNSTYRVVSVLTVLHQDWLNGKEYKCKVSNKALPAPIEKTISKAKGQPREPQVYTLPPSRDELTKNQVSLTCLVKGFYPSDIAVEWESNGQPENNYKTTPPVLDSDGSFFLYSKLTVDKSRWQQGNVFSCSVMHEALHNHYTQKSLSLSPGK

SEQ ID NO: 299 - protein, 449 aa, artificial sequence
  G4_20 IgG1 antibody heavy chain sequence
QVQLVESGAEVKKPGASVKVSCKASGGTFSSYAISWVRQAPGQGLEWMGGIIPIFGTANYAQKFQGRVTITVDKSTRTAYMELSSLRSKDTAVYYCARGNSRSDAFDIWGQGTMVTVSSASTKGPSVFPLAPSSKSTSGGTAALGCLVKDYFPEPVTVSWNSGALTSGVHTFPAVLQSSGLYSLSSVVTVPSSSLGTQTYICNVNHKPSNTKVDKKVEPKSCDKTHTCPPCPAPELLGGPSVFLFPPKPKDTLMISRTPEVTCVVVDVSHEDPEVKFNWYVDGVEVHNAKTKPREEQYNSTYRVVSVLTVLHQDWLNGKEYKCKVSNKALPAPIEKTISKAKGQPREPQVYTLPPSRDELTKNQVSLTCLVKGFYPSDIAVEWESNGQPENNYKTTPPVLDSDGSFFLYSKLTVDKSRWQQGNVFSCSVMHEALHNHYTQKSLSLSPGK

SEQ ID NO: 300 - protein, 450 aa, artificial sequence
  G4_22 IgG1 antibody heavy chain sequence
QVQLVESGGGLVQPGGSLRLSCAASGFTFSTYAMSWVRQAPGKGLEWVSTVSGSGGTTYYADSVKGRFTISRDNSKNTLYLQMNSLRAEDTAVYYCAKDSTAVTDWFDPWGRGTLVTVSSASTKGPSVFPLAPSSKSTSGGTAALGCLVKDYFPEPVTVSWNSGALTSGVHTFPAVLQSSGLYSLSSVVTVPSSSLGTQTYICNVNHKPSNTKVDKKVEPKSCDKTHTCPPCPAPELLGGPSVFLFPPKPKDTLMISRTPEVTCVVVDVSHEDPEVKFNWYVDGVEVHNAKTKPREEQYNSTYRVVSVLTVLHQDWLNGKEYKCKVSNKALPAPIEKTISKAKGQPREPQVYTLPPSRDELTKNQVSLTCLVKGFYPSDIAVEWESNGQPENNYKTTPPVLDSDGSFFLYSKLTVDKSRWQQGNVFSCSVMHEALHNHYTQKSLSLSPGK

SEQ ID NO: 301 - protein, 450 aa, artificial sequence
  G4_23 IgG1 antibody heavy chain sequence
EVQLVESGGGVVQPGRSLRLSCAASGFTFSSYGMHWVRQAPGKGLEWVAVIWYDGSNKYYADSVKGRFTISRDNSKNTLYLQMNSLRAEDTAVYYCARGEVAALYYFDYWGQGTLVTVSSASTKGPSVFPLAPSSKSTSGGTAALGCLVKDYFPEPVTVSWNSGALTSGVHTFPAVLQSSGLYSLSSVVTVPSSSLGTQTYICNVNHKPSNTKVDKKVEPKSCDKTHTCPPCPAPELLGGPSVFLFPPKPKDTLMISRTPEVTCVVVDVSHEDPEVKFNWYVDGVEVHNAKTKPREEQYNSTYRVVSVLTVLHQDWLNGKEYKCKVSNKALPAPIEKTISKAKGQPREPQVYTLPPSRDELTKNQVSLTCLVKGFYPSDIAVEWESNGQPENNYKTTPPVLDSDGSFFLYSKLTVDKSRWQQGNVFSCSVMHEALHNHYTQKSLSLSPGK

SEQ ID NO: 302 - protein, 452 aa, artificial sequence
  G4_24 IgG1 antibody heavy chain sequence
QVQLQQSGPGLVKPSQTLSLTCAISGASVSSNSVAWNWIRQSPSRGLEWLGRTYYRSRWYNDYALSVKSRIIINPDTSKNQFSLQLNSVTPEDTAVYYCARDWSSTRSFDYWGRGTLVTVSSASTKGPSVFPLAPSSKSTSGGTAALGCLVKDYFPEPVTVSWNSGALTSGVHTFPAVLQSSGLYSLSSVVTVPSSSLGTQTYICNVNHKPSNTKVDKKVEPKSCDKTHTCPPCPAPELLGGPSVFLFPPKPKDTLMISRTPEVTCVVVDVSHEDPEVKFNWYVDGVEVHNAKTKPREEQYNSTYRVVSVLTVLHQDWLNGKEYKCKVSNKALPAPIEKTISKAKGQPREPQVYTLPPSRDELTKNQVSLTCLVKGFYPSDIAVEWESNGQPENNYKTTPPVLDSDGSFFLYSKLTVDKSRWQQGNVFSCSVMHEALHNHYTQKSLSLSPGK

SEQ ID NO: 303 - protein, 453 aa, artificial sequence
  G4_25 IgG1 antibody heavy chain sequence
EVQLVESGAEVKKPGSSVKVSCKASGGTFSSYAISWVRQAPGQGLEWMGGIIPIFGTANYAQKFQGRVTITADKSTSTAYMELSSLRSEDTAVYYCARSLRDGYNYIGSLGYWGQGTLVTVSSASTKGPSVFPLAPSSKSTSGGTAALGCLVKDYFPEPVTVSWNSGALTSGVHTFPAVLQSSGLYSLSSVVTVPSSSLGTQTYICNVNHKPSNTKVDKKVEPKSCDKTHTCPPCPAPELLGGPSVFLFPPKPKDTLMISRTPEVTCVVVDVSHEDPEVKFNWYVDGVEVHNAKTKPREEQYNSTYRVVSVLTVLHQDWLNGKEYKCKVSNKALPAPIEKTISKAKGQPREPQVYTLPPSRDELTKNQVSLTCLVKGFYPSDIAVEWESNGQPENNYKTTPPVLDSDGSFFLYSKLTVDKSRWQQGNVFSCSVMHEALHNHYTQKSLSLSPGK

SEQ ID NO: 304 - protein, 450 aa, artificial sequence
  G4_26 IgG1 antibody heavy chain sequence
QVQLVQSGAEVKKPGSSVKVSCKASGGTFSSYAISWVRQAPGQGLEWMGGIIPIFGTANYAQKFQGRVTITADESTSTAYMELSSLRSEDTAVYYCASSRGSGWFPLGYWGQGTLVTVSSASTKGPSVFPLAPSSKSTSGGTAALGCLVKDYFPEPVTVSWNSGALTSGVHTFPAVLQSSGLYSLSSVVTVPSSSLGTQTYICNVNHKPSNTKVDKKVEPKSCDKTHTCPPCPAPELLGGPSVFLFPPKPKDTLMISRTPEVTCVVVDVSHEDPEVKFNWYVDGVEVHNAKTKPREEQYNSTYRVVSVLTVLHQDWLNGKEYKCKVSNKALPAPIEKTISKAKGQPREPQVYTLPPSRDELTKNQVSLTCLVKGFYPSDIAVEWESNGQPENNYKTTPPVLDSDGSFFLYSKLTVDKSRWQQGNVFSCSVMHEALHNHYTQKSLSLSPGK

SEQ ID NO: 305 - protein, 452 aa, artificial sequence
  G4_27 IgG1 antibody heavy chain sequence
QVQLVQSGAEVKKPGESLKISCKSSGYSFTSYWIGWVRQMPGKGLEWMGIIYPGDSDTRYSPSFQGQVTFSADESISTAYLQWSSLKASDTAMYYCARHGAYGDYPDTFDIWGQGTLVTVSSASTKGPSVFPLAPSSKSTSGGTAALGCLVKDYFPEPVTVSWNSGALTSGVHTFPAVLQSSGLYSLSSVVTVPSSSLGTQTYICNVNHKPSNTKVDKKVEPKSCDKTHTCPPCPAPELLGGPSVFLFPPKPKDTLMISRTPEVTCVVVDVSHEDPEVKFNWYVDGVEVHNAKTKPREEQYNSTYRVVSVLTVLHQDWLNGKEYKCKVSNKALPAPIEKTISKAKGQPREPQVYTLPPSRDELTKNQVSLTCLVKGFYPSDIAVEWESNGQPENNYKTTPPVLDSDGSFFLYSKLTVDKSRWQQGNVFSCSVMHEALHNHYTQKSLSLSPGK

SEQ ID NO: 306 - protein, 455 aa, artificial sequence
  G4_28 IgG1 antibody heavy chain sequence
QVQLVESGGGLVQPGGSLRLSCAASGFTFDDYAMHWVRQAPGKGLEWVSGISAGGGSTNYAGSVKGRFTVSRDTSKNTLYLQMNSLRAEDTAVYYCVKSYVDTAMRYYYYYMDVWGQGTMVTVSSASTKGPSVFPLAPSSKSTSGGTAALGCLVKDYFPEPVTVSWNSGALTSGVHTFPAVLQSSGLYSLSSVVTVPSSSLGTQTYICNVNHKPSNTKVDKKVEPKSCDKTHTCPPCPAPELLGGPSVFLFPPKPKDTLMISRTPEVTCVVVDVSHEDPEVKFNWYVDGVEVHNAKTKPREEQYNSTYRVVSVLTVLHQDWLNGKEYKCKVSNKALPAPIEKTISKAKGQPREPQVYTLPPSRDELTKNQVSLTCLVKGFYPSDIAVEWESNGQPENNYKTTPPVLDSDGSFFLYSKLTVDKSRWQQGNVFSCSVMHEALHNHYTQKSLSLSPGK

SEQ ID NO: 307 - protein, 216 aa, artificial sequence
  G4_1 IgG1 antibody light chain sequence
ASDIQMTQSPSSLSASVGDRVTITCQASQDISNYLNWYQQKPGKAPKLLIYDASNLETGVPSRFSGSGSGTDFTLTISSLQPEDFATYYCQQSYSTPVTFGPGTKVEIKRTAAAPSVFIFPPSDEQLKSGTASVVCLLNNFYPREAKVQWKVDNALQSGNSQESVTEQDSKDSTYSLSSTLTLSKADYEKHKLYACEVTHQGLSSPVTKSFNRGEC

SEQ ID NO: 308 - protein, 216 aa, artificial sequence
  G4_2 IgG1 antibody light chain sequence
ASDIQMTQSPSSLSASVGDRVTITCQASQDISNYLNWYQQKPGKAPKLLIYAASSLQSGVPSRFSGSGSGTDFTLTISGLQPEDFATYYCLEDYNYLWTFGQGTKLEIKRTAAAPSVFIFPPSDEQLKSGTASVVCLLNNFYPREAKVQWKVDNALQSGNSQESVTEQDSKDSTYSLSSTLTLSKADYEKHKLYACEVTHQGLSSPVTKSFNRGEC

SEQ ID NO: 309 - protein, 216 aa, artificial sequence
  G4_3 IgG1 antibody light chain sequence
ASDIQMTQSPSSLSASVGDRVTITCQASQDISNYLNWYQQKPGKAPKLLIYDASNLETGVPSRFSGSGSGTDFTLTISSLQPEDFATYFCQQSYSTPQTFGQGTKVDIKRTAAAPSVFIFPPSDEQLKSGTASVVCLLNNFYPREAKVQWKVDNALQSGNSQESVTEQDSKDSTYSLSSTLTLSKADYEKHKLYACEVTHQGLSSPVTKSFNRGEC

SEQ ID NO: 310 - protein, 222 aa, artificial sequence
  G4_4 IgG1 antibody light chain sequence
ASDIVMTQSPDSLAVSLGERATINCKSSQSVLSSSNNNNYLAWYQQRPGQPPKLLFYWASTRESGVPDRFSGSGSGTSFTLTITSLQAEDVAVYYCQQYYSTPLTFGGGTKLEIKRTAAAPSVFIFPPSDEQLKSGTASVVCLLNNFYPREAKVQWKVDNALQSGNSQESVTEQDSKDSTYSLSSTLTLSKADYEKHKLYACEVTHQGLSSPVTKSFNRGEC

SEQ ID NO: 311 - protein, 216 aa, artificial sequence
  G4_5 IgG1 antibody light chain sequence
ASDIQMTQSPSSLSASVGDRVTITCRASQSISSYLNWYQQKPGKAPKLLIYAASSLQSGVPSRFSGSGSGTDFTLTISSLQPEDFATYYCQQSYSTPYTFGQGTKVEIKRTAAAPSVFIFPPSDEQLKSGTASVVCLLNNFYPREAKVQWKVDNALQSGNSQESVTEQDSKDSTYSLSSTLTLSKADYEKHKLYACEVTHQGLSSPVTKSFNRGEC

SEQ ID NO: 312 - protein, 216 aa, artificial sequence
  G4_6 IgG1 antibody light chain sequence
ASDIQMTQSPSSLSASVGDRVTITCRASQSISTYLNWYQQKPGKAPKLLIYAASSLQSGVPSRFSGSGSGTDFTLTISSPQPEDFATYYCQQSYSTPYTFGQGTKVEIKRTAAAPSVFIFPPSDEQLKSGTASVVCLLNNFYPREAKVQWKVDNALQSGNSQESVTEQDSKDSTYSLSSTLTLSKADYEKHKLYACEVTHQGLSSPVTKSFNRGEC

SEQ ID NO: 313 - protein, 221 aa, artificial sequence
  G4_7 IgG1 antibody light chain sequence
ASDIVMTQSPLSLPVTPGEPASISCRSSQSLLHSNRFNYLDWYLQKPGQSPQLLIYLGSNRASGVPDRFSGSGSGTDFTLKISRVEAEDVGVYYCMQGLQTPYTFGQGTKVDIKRTAAAPSVFIFPPSDEQLKSGTASVVCLLNNFYPREAKVQWKVDNALQSGNSQESVTEQDSKDSTYSLSSTLTLSKADYEKHKLYACEVTHQGLSSPVTKSFNRGEC

SEQ ID NO: 314 - protein, 221 aa, artificial sequence
  G4_10 IgG1 antibody light chain sequence
ASDIVMTQPPLSLPVTLGHPASISCKSSQSLEYSDGNTYLNWFQQRPGQSPRRLIYKVSNRDSGAPDRFSGSGSGTDFTLEISRVEAEDVGVYYCMQGTLWPPTFGQGTKVDIKRTAAAPSVFIFPPSDEQLKSGTASVVCLLNNFYPREAKVQWKVDNALQSGNSQESVTEQDSKDSTYSLSSTLTLSKADYEKHKLYACEVTHQGLSSPVTKSFNRGEC

SEQ ID NO: 315 - protein, 216 aa, artificial sequence
  G4_12 IgG1 antibody light chain sequence
ASQSVLTQPASVSGSPGQSITISCTGTSSDVGGYNFVSWYQQHPGKAPKLMIYEVTNRPSGVPDRFSGSKSGNTASLTISGLQAEDEADYYCSSHASPRVFGTGTKVTVLGQPAAAPSVTLFPPSSEELQANKATLVCLISDFYPGAVTVAWKADSSPVKAGVETTTPSKQSNNKYAASSYLSLTPEQWKSHRSYSCQVTHEGSTVEKTVAPTECS

SEQ ID NO: 316 - protein, 219 aa, artificial sequence
  G4_13 IgG1 antibody light chain sequence
ASNFMLTQPHSVSESPGKTVTISCTRSSGSIASNYVQWYQQRPGSSPSTVIYEDNQRPSGVPDRFSGSIDSSSNSASLTISGLRTEDEADYYCQSYDSSIYVVFGGGTKLTVLGQPAAAPSVTLFPPSSEELQANKATLVCLISDFYPGAVTVAWKADSSPVKAGVETTTPSKQSNNKYAASSYLSLTPEQWKSHRSYSCQVTHEGSTVEKTVAPTECS

SEQ ID NO: 317 - protein, 219 aa, artificial sequence
  G4_14 IgG1 antibody light chain sequence
ASNFMLTQPHSVSESPGKTVTISCTRSRGSIAGNYVHWYQQRPGRAPTTVIYRDKERPSGVPDRISGSIDSSSNSASLTISGLKTEDEADYYCQSYDSSTHVVFGGGTKLTVLGQPAAAPSVTLFPPSSEELQANKATLVCLISDFYPGAVTVAWKADSSPVKAGVETTTPSKQSNNKYAASSYLSLTPEQWKSHRSYSCQVTHEGSTVEKTVAPTECS

SEQ ID NO: 318 - protein, 216 aa, artificial sequence
  G4_15 IgG1 antibody light chain sequence
ASQSALTQPASVSGSPGQSITISCTGTSSDVGGYNYVSWYQQHPGKAPKLMIYDVSNRPSGVSNRFSGSKSGNTASLTISGLQAEDEADYYCSSYGSGSVFGTGTKLTVLGQPAAAPSVTLFPPSSEELQANKATLVCLISDFYPGAVTVAWKADSSPVKAGVETTTPSKQSNNKYAASSYLSLTPEQWKSHRSYSCQVTHEGSTVEKTVAPTECS

SEQ ID NO: 319 - protein, 218 aa, artificial sequence
  G4_16 IgG1 antibody light chain sequence
ASQSVLTQPPSASGSPGQSVTFSCTGTSSDIGAFNSVSWYQQHPGKAPKLLIYEITKRPSGVPDRFSGSKSGNTASLTISVLQAEDEADYYCTSYAGSNTLIFGGGTKVTVLGQPAAAPSVTLFPPSSEELQANKATLVCLISDFYPGAVTVAWKADSSPVKAGVETTTPSKQSNNKYAASSYLSLTPEQWKSHRSYSCQVTHEGSTVEKTVAPTECS

SEQ ID NO: 320 - protein, 216 aa, artificial sequence
  G4_18 IgG1 antibody light chain sequence
ASSYELTQPPSVTESPGQTARITCSGDALAKQYAYWYQQKPGQAPVLVIYRDSERPSEIPERFSGSSSGTTVTLTISGVQAEDEADYYCQSADSSGTYTVFGGGTKLTVLGQPAAAPSVTLFPPSSEELQANKATLVCLISDFYPGAVTVAWKADSSPVKAGVETTTPSKQSNNKYAASSYLSLTPEQWKSHRSYSCQVTHEGSTVEKTVAPTECS

SEQ ID NO: 321 - protein, 219 aa, artificial sequence
  G4_19 IgG1 antibody light chain sequence
ASNFMLTQPHSVSESPGKTVTISCTRSSGSIASNYVQWYQQRPGSPPITLIYDDDQRPSGVPHRFSGSIDTSSNPASLTISGLKTEDEADYYCQSYDSSNHVVFGGGTKLTVLGQPAAAPSVTLFPPSSEELQANKATLVCLISDFYPGAVTVAWKADSSPVKAGVETTTPSKQSNNKYAASSYLSLTPEQWKSHRSYSCQVTHEGSTVEKTVAPTECS

SEQ ID NO: 322 - protein, 214 aa, artificial sequence
  G4_20 IgG1 antibody light chain sequence
ASSYELTHPPSVSVSPGQTASITCSGDKLGDKFVSWYHQKPGQSPVLVIYQDSKRPSGIPERFSGSNSGNTATLTISGTRAMDEADYYCQAWDSSTVVFGGGTKLTVLGQPAAAPSVTLFPPSSEELQANKATLVCLISDFYPGAVTVAWKADSSPVKAGVETTTPSKQSNNKYAASSYLSLTPEQWKSHRSYSCQVTHEGSTVEKTVAPTECS

SEQ ID NO: 323 - protein, 216 aa, artificial sequence
  G4_22 IgG1 antibody light chain sequence
ASDIQMTQSPSSLSASVGDRVTITCQASQDISNYLNWYQQKPGKAPKLLIYAASSLQSGVPSRFSVSGSGTDFTLTISNLQPEDFATYYCQQSYSIPWTFGQGTKVEIKRTAAAPSVFIFPPSDEQLKSGTASVVCLLNNFYPREAKVQWKVDNALQSGNSQESVTEQDSKDSTYSLSSTLTLSKADYEKHKLYACEVTHQGLSSPVTKSFNRGEC

SEQ ID NO: 324 - protein, 216 aa, artificial sequence
  G4_23 IgG1 antibody light chain sequence
ASDIQMTQSPSSLSASVGDRVTITCRASQGISNSLAWYQQKPGKAPKLLLYAASRLESGVPSRFSGSGSGTDYTLTISSLQPEDFATYYCQQYYSTPRTFGGGTKLEIKRTAAAPSVFIFPPSDEQLKSGTASVVCLLNNFYPREAKVQWKVDNALQSGNSQESVTEQDSKDSTYSLSSTLTLSKADYEKHKLYACEVTHQGLSSPVTKSFNRGEC

SEQ ID NO: 325 - protein, 222 aa, artificial sequence
  G4_24 IgG1 antibody light chain sequence
ASDIVMTQSPDSLAVSLGERATINCKSSQSVLYSSNNKNYLAWYQQKPGQPPKLLISWASTRESGVPDRFSGSGSGTDFTLTINSLQSEDVAIYYCQQYYSTPPTFGQGTKLEIKRTAAAPSVFIFPPSDEQLKSGTASVVCLLNNFYPREAKVQWKVDNALQSGNSQESVTEQDSKDSTYSLSSTLTLSKADYEKHKLYACEVTHQGLSSPVTKSFNRGEC

SEQ ID NO: 326 - protein, 216 aa, artificial sequence
  G4_25 IgG1 antibody light chain sequence
ASQSALTQPRSVSGSPGQSVTISCTGTSSDVGGYNYVSWYQQHPGKAPKLMIYEVSNRPSGVSNRFSGSKSGNTASLTISGLQAEDEADYYCSSYGSGSVFGTGTKLTVLGQPAAAPSVTLFPPSSEELQANKATLVCLISDFYPGAVTVAWKADSSPVKAGVETTTPSKQSNNKYAASSYLSLTPEQWKSHRSYSCQVTHEGSTVEKTVAPTECS

SEQ ID NO: 327 - protein, 216 aa, artificial sequence
  G4_26 IgG1 antibody light chain sequence
ASQSGLTQPASVSGSPGQSITISCTGTSSDVGSYNLVSWYQQHPGKAPKLMIYEVSKRPSGVSNRFSGSKSGNTASLTISGLQAEDEADYYCSSFGSGSIFGTGTKLTVLGQPAAAPSVTLFPPSSEELQANKATLVCLISDFYPGAVTVAWKADSSPVKAGVETTTPSKQSNNKYAASSYLSLTPEQWKSHRSYSCQVTHEGSTVEKTVAPTECS

SEQ ID NO: 328 - protein, 216 aa, artificial sequence
  G4_27 IgG1 antibody light chain sequence
ASSYELTQDPAVSVALGQTVSITCQGDSLRNFYANWYQQKPGQAPVLVIYGKNNRPSGIPDRFSGSSSGNTASLTITGAQAEDEADYYCNSRDSSGNHLVFGGGTQLTVLGQPAAAPSVTLFPPSSEELQANKATLVCLISDFYPGAVTVAWKADSSPVKAGVETTTPSKQSNNKYAASSYLSLTPEQWKSHRSYSCQVTHEGSTVEKTVAPTECS

SEQ ID NO: 329 - protein, 214 aa, artificial sequence
  G4_28 IgG1 antibody light chain sequence
ASSYELTQDPAVSVALGQTVTITCQGDSLRNYYASWYRQKPGQTPVLVVYGKNNRPSGIPDRFSVSASGNTASLTITGAQAEDEGDYYCNSRDSSGVVFGGGTKVTVLGQPAAAPSVTLFPPSSEELQANKATLVCLISDFYPGAVTVAWKADSSPVKAGVETTTPSKQSNNKYAASSYLSLTPEQWKSHRSYSCQVTHEGSTVEKTVAPTECS

SEQ ID NO: 330 - protein, 107 aa, artificial sequence [sequence omitted]

SEQ ID NO: 331 - protein, 106 aa, artificial sequence
  Human Lambda light constant sequence (IGLC2 without cloning artefacts)
GQPKAAPSVTLFPPSSEELQANKATLVCLISDFYPGAVTVAWKADSSPVKAGVETTTPSKQSNNKYAASSYLSLTPEQWKSHRSYSCQVTHEGSTVEKTVAPTECS

SEQ ID NO: 332 - protein, 330 aa, artificial sequence [sequence omitted]

SEQ ID NO: 333 - protein, 330 aa, artificial sequence
  Human IgG1 constant domain with LAGA substitution
ASTKGPSVFPLAPSSKSTSGGTAALGCLVKDYFPEPVTVSWNSGALTSGVHTFPAVLQSSGLYSLSSVVTVPSSSLGTQTYICNVNHKPSNTKVDKKVEPKSCDKTHTCPPCPAPELAGAPSVFLFPPKPKDTLMISRTPEVTCVVVDVSHEDPEVKFNWYVDGVEVHNAKTKPREEQYNSTYRVVSVLTVLHQDWLNGKEYKCKVSNKALPAPIEKTISKAKGQPREPQVYTLPPSRDELTKNQVSLTCLVKGFYPSDIAVEWESNGQPENNYKTTPPVLDSDGSFFLYSKLTVDKSRWQQGNVFSCSVMHEALHNHYTQKSLSLSPGK

SEQ ID NO: 334 - protein, 99 aa, Homo sapiens
  Human TRGV4
SSNLEGRTKSVIRQTGSSAEITCDLAEGSTGYIHWYLHQEGKAPQRLLYYDSYTSSVVLESGISPGKYDTYGSTRKNLRMILRNLIENDSGVYYCATWD

SEQ ID NO: 335 - protein, 99 aa, Homo sapiens
  Human TRGV2
SSNLEGRTKSVIRQTGSSAEITCDLAEGSNGYIHWYLHQEGKAPQRLQYYDSYNSKVVLESGVSPGKYYTYASTRNNLRLILRNLIENDSGVYYCATWD

SEQ ID NO: 336 - protein, 99 aa, Homo sapiens
  Human TRGV8
SSNLEGRTKSVTRPTGSSAVITCDLPVENAVYTHWYLHQEGKAPQRLLYYDSYNSRVVLESGISREKYHTYASTGKSLKFILENLIERDSGVYYCATWD

SEQ ID NO: 337 - protein, 95 aa, Homo sapiens
  Human TRDV1
AQKVTQAQSSVSMPVRKAVTLNCLYETSWWSYYIFWYKQLPSKEMIFLIRQGSDEQNAKSGRYSVNFKKAAKSVALTISALQLEDSAKYFCALGE

SEQ ID NO: 338 - protein, 96 aa, Homo sapiens
  Human TRDV2
AIELVPEHQTVPVSIGVPATLRCSMKGEAIGNYYINWYRKTQGNTITFIYREKDIYGPGFKDNFQGDIDIAKNLAVLKILAPSERDEGSYYCACDT